European Patent Specification EP 3 712 173 B1, published July 12, 2023. Title: PDGF RECEPTOR BETA BINDING POLYPEPTIDES. Applicant: X-BODY, INC. The sequence listing filed with the application follows.

SEQUENCE LISTING (508 sequences)

SEQ ID NO: 1 - protein, 7 aa, Artificial Sequence
  Synthetic Heavy chain CDR
HGGDRSY

SEQ ID NO: 2 - protein, 17 aa, Artificial Sequence
  Synthetic Heavy chain CDR
GIIPIFGTANYAQKFQG

SEQ ID NO: 3 - protein, 17 aa, Artificial Sequence
  Synthetic Heavy chain CDR
GILPILKTPNYAQRFQG

SEQ ID NO: 4 - protein, 17 aa, Artificial Sequence
  Synthetic Heavy chain CDR, clone: C05
GVLPILKTPNYAQRFQG

SEQ ID NO: 5 - protein, 17 aa, Artificial Sequence
  Synthetic Heavy chain CDR, clone: E2
WINPNSGNTGYAQKFQG

SEQ ID NO: 6 - protein, 17 aa, Artificial Sequence
  Synthetic Heavy chain CDR, clone: A3
WINPNSGGTYFAQKFQG

SEQ ID NO: 7 - protein, 17 aa, Artificial Sequence
  Synthetic Heavy chain CDR, clone: F10
WINPDSGGTYFAQKFQG

SEQ ID NO: 8 - protein, 17 aa, Artificial Sequence
  Synthetic Heavy chain CDR, clone: C12
WMNPDSGGTIYAQKFQG

SEQ ID NO: 9 - protein, 17 aa, Artificial Sequence
  Synthetic Heavy chain CDR, clone: H2
WLNPNSGDTHSAQKFQG

SEQ ID NO: 10 - protein, 17 aa, Artificial Sequence
  Synthetic Heavy chain CDR, clone: B1
WINPNNGNTTYAQKFQG

SEQ ID NO: 11 - protein, 17 aa, Artificial Sequence
  Synthetic Heavy chain CDR, clone: H1
WINPNSGGTNSAPKFQG

SEQ ID NO: 12 - protein, 17 aa, Artificial Sequence
  Synthetic Heavy chain CDR, clone: E6
WINPNSGGTNYAQKFQG

SEQ ID NO: 13 - protein, 17 aa, Artificial Sequence
  Synthetic Heavy chain CDR
WIVVGSGNTNYAQKFQE

SEQ ID NO: 14 - protein, 17 aa, Artificial Sequence
  Synthetic Heavy chain CDR
VINTGVGSTNYAQKFQG

SEQ ID NO: 15 - protein, 17 aa, Artificial Sequence
  Synthetic Heavy chain CDR, clone: H3
LSNPSGDYTVYAPKFQG

SEQ ID NO: 16 - protein, 17 aa, Artificial Sequence
  Synthetic Heavy chain CDR, clone: B4
LSNPSGDYTVYAPKLQG

SEQ ID NO: 17 - protein, 17 aa, Artificial Sequence
  Synthetic Heavy chain CDR, clone: D06
VISYDGSNKYYADSVKG

SEQ ID NO: 18 - protein, 17 aa, Artificial Sequence
  Synthetic Heavy chain CDR, clone: F3
WISADNGNTNYAQKFQE

SEQ ID NO: 19 - protein, 17 aa, Artificial Sequence
  Synthetic Heavy chain CDR, clone: A12
WISADNGNTKYAQKFQD

SEQ ID NO: 20 - protein, 17 aa, Artificial Sequence
  Synthetic Heavy chain CDR, clone: G3
GFDPEDGETIYAQKFQG

SEQ ID NO: 21 - protein, 17 aa, Artificial Sequence
  Synthetic Heavy chain CDR, clone: G12
GIIPVSGTPNYAQKFQG

SEQ ID NO: 22 - protein, 17 aa, Artificial Sequence
  Synthetic Heavy chain CDR, clone: E9
ITYPADSTTVYSPSFQG

SEQ ID NO: 23 - protein, 17 aa, Artificial Sequence
  Synthetic Heavy chain CDR, clone: E11
RINNDGSSTSYADSVKG

SEQ ID NO: 24 - protein, 17 aa, Artificial Sequence
  Synthetic Heavy chain CDR, clone: C08
RISIDGTTTTYADSVQG

SEQ ID NO: 25 - protein, 17 aa, Artificial Sequence
  Synthetic Heavy chain CDR, clone: XB2708
FILFDGNNKYYADSVKG

SEQ ID NO: 26 - protein, 17 aa, Artificial Sequence
  Synthetic Heavy chain CDR, clone: D03
RINADGTSTAYAESVKG

SEQ ID NO: 27 - protein, 16 aa, Artificial Sequence
  Synthetic Heavy chain CDR, clone: A10
LIYSDGSTYYADSVKG

SEQ ID NO: 28 - protein, 17 aa, Artificial Sequence
  Synthetic Heavy chain CDR, clone: C09
AIDGSGGTTYYAGSVKG

SEQ ID NO: 29 - protein, 17 aa, Artificial Sequence
  Synthetic Heavy chain CDR, clone: A06
HISNDGSITRYADSVKG

SEQ ID NO: 30 - protein, 17 aa, Artificial Sequence
  Synthetic Heavy chain CDR, clone: C05
RIKTDGSSTSYADSVKG

SEQ ID NO: 31 - protein, 17 aa, Artificial Sequence
  Synthetic Heavy chain CDR, clone: H01
RISSDGSTTAYADSVRG

SEQ ID NO: 32 - protein, 17 aa, Artificial Sequence
  Synthetic Heavy chain CDR, clone: G07
RISSDGSSTAYADSVKG

SEQ ID NO: 33 - protein, 5 aa, Artificial Sequence
  Synthetic Heavy chain CDR
SYAIS

SEQ ID NO: 34 - protein, 5 aa, Artificial Sequence
  Synthetic Heavy chain CDR, clone: G2
GYAIS

SEQ ID NO: 35 - protein, 5 aa, Artificial Sequence
  Synthetic Heavy chain CDR
RHAIS

SEQ ID NO: 36 - protein, 5 aa, Artificial Sequence
  Synthetic Heavy chain CDR
DYYIQ

SEQ ID NO: 37 - protein, 5 aa, Artificial Sequence
  Synthetic Heavy chain CDR, clone: H2
AYYIQ

SEQ ID NO: 38 - protein, 5 aa, Artificial Sequence
  Synthetic Heavy chain CDR
DYYIH

SEQ ID NO: 39 - protein, 5 aa, Artificial Sequence
  Synthetic Heavy chain CDR, clone: H1
DYHLH

SEQ ID NO: 40 - protein, 5 aa, Artificial Sequence
  Synthetic Heavy chain CDR, clone: E6
DYYLH

SEQ ID NO: 41 - protein, 5 aa, Artificial Sequence
  Synthetic Heavy chain CDR, clone: A1
SSAVQ

SEQ ID NO: 42 - protein, 5 aa, Artificial Sequence
  Synthetic Heavy chain CDR, clone: H7
SSAMQ

SEQ ID NO: 43 - protein, 5 aa, Artificial Sequence
  Synthetic Heavy chain CDR, clone: B2
NYQVQ

SEQ ID NO: 44 - protein, 5 aa, Artificial Sequence
  Synthetic Heavy chain CDR, clone: A7
NYPVQ

SEQ ID NO: 45 - protein, 5 aa, Artificial Sequence
  Synthetic Heavy chain CDR
NSFMQ

SEQ ID NO: 46 - protein, 5 aa, Artificial Sequence
  Synthetic Heavy chain CDR
SYGMH

SEQ ID NO: 47 - protein, 5 aa, Artificial Sequence
  Synthetic Heavy chain CDR
SHGMS

SEQ ID NO: 48 - protein, 5 aa, Artificial Sequence
  Synthetic Heavy chain CDR, clone: G3
ELSMH

SEQ ID NO: 49 - protein, 5 aa, Artificial Sequence
  Synthetic Heavy chain CDR, clone: H12
DNYVH

SEQ ID NO: 50 - protein, 5 aa, Artificial Sequence
  Synthetic Heavy chain CDR, clone: G12
AYPIS

SEQ ID NO: 51 - protein, 5 aa, Artificial Sequence
  Synthetic Heavy chain CDR, clone: C06
GHYIH

SEQ ID NO: 52 - protein, 5 aa, Artificial Sequence
  Synthetic Heavy chain CDR, clone: C11
NDYIH

SEQ ID NO: 53 - protein, 5 aa, Artificial Sequence
  Synthetic Heavy chain CDR, clone: F08
SSYIH

SEQ ID NO: 54 - protein, 5 aa, Artificial Sequence
  Synthetic Heavy chain CDR, clone: E9
NYWIG

SEQ ID NO: 55 - protein, 5 aa, Artificial Sequence
  Synthetic Heavy chain CDR, clone: E11
SYWMH

SEQ ID NO: 56 - protein, 5 aa, Artificial Sequence
  Synthetic Heavy chain CDR, clone: C08
AFWMH

SEQ ID NO: 57 - protein, 5 aa, Artificial Sequence
  Synthetic Heavy chain CDR, clone: D03
NDWMH

SEQ ID NO: 58 - protein, 5 aa, Artificial Sequence
  Synthetic Heavy chain CDR, clone: A10
DYAMN

SEQ ID NO: 59 - protein, 5 aa, Artificial Sequence
  Synthetic Heavy chain CDR, clone: C09
NNAMS

SEQ ID NO: 60 - protein, 5 aa, Artificial Sequence
  Synthetic Heavy chain CDR, clone: A06
GHWMH

SEQ ID NO: 61 - protein, 5 aa, Artificial Sequence
  Synthetic Heavy chain CDR, clone: C05
SNWMH

SEQ ID NO: 62 - protein, 5 aa, Artificial Sequence
  Synthetic Heavy chain CDR
SDWMH

SEQ ID NO: 63 - protein, 9 aa, Artificial Sequence
  Synthetic Light chain CDR, clone: B10
HQSSSLPWT

SEQ ID NO: 64 - protein, 9 aa, Artificial Sequence
  Synthetic Light chain CDR, clone: H10
HQSSSLPHT

SEQ ID NO: 65 - protein, 11 aa, Artificial Sequence
  Synthetic Light chain CDR, clone: F10
RASQSIGSGLH

SEQ ID NO: 66 - protein, 9 aa, Artificial Sequence
  Synthetic Light chain CDR, clone: B12
HQTSSLPLT

SEQ ID NO: 67 - protein, 9 aa, Artificial Sequence
  Synthetic Light chain CDR, clone: B11
QQYGSSPWT

SEQ ID NO: 68 - protein, 9 aa, Artificial Sequence
  Synthetic Light chain CDR, clone: E7
QQYGSSPQT

SEQ ID NO: 69 - protein, 10 aa, Artificial Sequence
  Synthetic Light chain CDR, clone: E8
QQYGSSPPYT

SEQ ID NO: 70 - protein, 9 aa, Artificial Sequence
  Synthetic Light chain CDR, clone: H8
QQYAGSPFT

SEQ ID NO: 71 - protein, 9 aa, Artificial Sequence
  Synthetic Light chain CDR, clone: H12
QQFGSSPWT

SEQ ID NO: 72 - protein, 9 aa, Artificial Sequence
  Synthetic Light chain CDR, clone: F8
QQYGSSPLT

SEQ ID NO: 73 - protein, 9 aa, Artificial Sequence
  Synthetic Light chain CDR, clone: D11
QQYGASPRT

SEQ ID NO: 74 - protein, 9 aa, Artificial Sequence
  Synthetic Light chain CDR, clone: G8
QQYGSALLT

SEQ ID NO: 75 - protein, 8 aa, Artificial Sequence
  Synthetic Light chain CDR, clone: H9
QQYGNSWT

SEQ ID NO: 76 - protein, 9 aa, Artificial Sequence
  Synthetic Light chain CDR, clone: H11
HQSRNLPFT

SEQ ID NO: 77 - protein, 9 aa, Artificial Sequence
  Synthetic Light chain CDR, clone: G12
HQSRSFPLT

SEQ ID NO: 78 - protein, 8 aa, Artificial Sequence
  Synthetic Light chain CDR, clone: E11
QQYETSWT

SEQ ID NO: 79 - protein, 8 aa, Artificial Sequence
  Synthetic Light chain CDR, clone: F12
RDGLNHLV

SEQ ID NO: 80 - protein, 11 aa, Artificial Sequence
  Synthetic Light chain CDR, clone: C8
GTWDSSLSVVI

SEQ ID NO: 81 - protein, 9 aa, Artificial Sequence
  Synthetic Light chain CDR, clone: A8
HQTGSFPYT

SEQ ID NO: 82 - protein, 10 aa, Artificial Sequence
  Synthetic Light chain CDR, clone: B8
LLSYSGPRVV

SEQ ID NO: 83 - protein, 9 aa, Artificial Sequence
  Synthetic Light chain CDR, clone: F7
QQSYRTPFS

SEQ ID NO: 84 - protein, 9 aa, Artificial Sequence
  Synthetic Light chain CDR, clone: B7
QVWDSSSVI

SEQ ID NO: 85 - protein, 11 aa, Artificial Sequence
  Synthetic Light chain CDR, clone: G9
KSRDSSAMRWV

SEQ ID NO: 86 - protein, 9 aa, Artificial Sequence
  Synthetic Light chain CDR, clone: A9
LLYFNPTRV

SEQ ID NO: 87 - protein, 7 aa, Artificial Sequence
  Synthetic Light chain CDR, clone: A11
GADHGRV

SEQ ID NO: 88 - protein, 8 aa, Artificial Sequence
  Synthetic Light chain CDR, clone: E12
QVWHSGVI

SEQ ID NO: 89 - protein, 8 aa, Artificial Sequence
  Synthetic Light chain CDR, clone: H7
HQSRSSHT

SEQ ID NO: 90 - protein, 11 aa, Artificial Sequence
  Synthetic Light chain CDR, clone: A10
QSFDVYSHEVV

SEQ ID NO: 91 - protein, 9 aa, Artificial Sequence
  Synthetic Light chain CDR, clone: C11
MQSTHFPFT

SEQ ID NO: 92 - protein, 9 aa, Artificial Sequence
  Synthetic Light chain CDR, clone: D10
QQYDSPPWT

SEQ ID NO: 93 - protein, 9 aa, Artificial Sequence
  Synthetic Light chain CDR, clone: D12
QQHDTSQWT

SEQ ID NO: 94 - protein, 9 aa, Artificial Sequence
  Synthetic Light chain CDR, clone: C7
MQGLHIPHT

SEQ ID NO: 95 - protein, 8 aa, Artificial Sequence
  Synthetic Light chain CDR, clone: D7
MQSTHQWT

SEQ ID NO: 96 - protein, 9 aa, Artificial Sequence
  Synthetic Light chain CDR, clone: C9
QQYDSYSRT

SEQ ID NO: 97 - protein, 8 aa, Artificial Sequence
  Synthetic Light chain CDR, clone: C12
QQSFSMRT

SEQ ID NO: 98 - protein, 8 aa, Artificial Sequence
  Synthetic Light chain CDR, clone: D8
QQYVNSRT

SEQ ID NO: 99 - protein, 8 aa, Artificial Sequence
  Synthetic Light chain CDR, clone: D9
QQYNDFFT

SEQ ID NO: 100 - protein, 8 aa, Artificial Sequence
  Synthetic Light chain CDR, clone: G7
MQATQFPS

SEQ ID NO: 101 - protein, 9 aa, Artificial Sequence
  Synthetic Light chain CDR, clone: G11
QQYGDSVFT

SEQ ID NO: 102 - protein, 9 aa, Artificial Sequence
  Synthetic Light chain CDR, clone: F9
QQSYSTPRT

SEQ ID NO: 103 - protein, 10 aa, Artificial Sequence
  Synthetic Light chain CDR, clone: E9
QESYSTLLYT

SEQ ID NO: 104 - protein, 11 aa, Artificial Sequence
  Synthetic Light chain CDR, clone: B1
QVWESGSEHYV

SEQ ID NO: 105 - protein, 11 aa, Artificial Sequence
  Synthetic Light chain CDR, clone: E6
QVWESTSDHPT

SEQ ID NO: 106 - protein, 11 aa, Artificial Sequence
  Synthetic Light chain CDR, clone: F3
QVWDSSSDHWV

SEQ ID NO: 107 - protein, 12 aa, Artificial Sequence
  Synthetic Light chain CDR, clone: H4
QVWDSSSGHRGV

SEQ ID NO: 108 - protein, 11 aa, Artificial Sequence
  Synthetic Light chain CDR, clone: H5
QVWDSATDHVV

SEQ ID NO: 109 - protein, 11 aa, Artificial Sequence
  Synthetic Light chain CDR, clone: B5
QVWDSDRHHVV

SEQ ID NO: 110 - protein, 11 aa, Artificial Sequence
  Synthetic Light chain CDR, clone: G6
QVWDINDDYAV

SEQ ID NO: 111 - protein, 11 aa, Artificial Sequence
  Synthetic Light chain CDR, clone: C1
QQYVSSPPMYT

SEQ ID NO: 112 - protein, 9 aa, Artificial Sequence
  Synthetic Light chain CDR, clone: F1
QQYVTYPLT

SEQ ID NO: 113 - protein, 9 aa, Artificial Sequence
  Synthetic Light chain CDR, clone: A3
QQYDSVPLT

SEQ ID NO: 114 - protein, 9 aa, Artificial Sequence
  Synthetic Light chain CDR, clone: B4
QQYEDLPSF

SEQ ID NO: 115 - protein, 9 aa, Artificial Sequence
  Synthetic Light chain CDR, clone: B6
QQYGSFPYS

SEQ ID NO: 116 - protein, 9 aa, Artificial Sequence
  Synthetic Light chain CDR, clone: F2
QQYQNPPFT

SEQ ID NO: 117 - protein, 9 aa, Artificial Sequence
  Synthetic Light chain CDR, clone: D3
QQYKTFPHT

SEQ ID NO: 118 - protein, 9 aa, Artificial Sequence
  Synthetic Light chain CDR, clone: G2
QQYHSYPYT

SEQ ID NO: 119 - protein, 9 aa, Artificial Sequence
  Synthetic Light chain CDR, clone: A4
QQYNNVLRT

SEQ ID NO: 120 - protein, 9 aa, Artificial Sequence
  Synthetic Light chain CDR, clone: G4
QQYNKWPTF

SEQ ID NO: 121 - protein, 10 aa, Artificial Sequence
  Synthetic Light chain CDR, clone: D5
QQYYNWPPWT

SEQ ID NO: 122 - protein, 9 aa, Artificial Sequence
  Synthetic Light chain CDR, clone: A1
QQRSNGVTF

SEQ ID NO: 123 - protein, 9 aa, Artificial Sequence
  Synthetic Light chain CDR, clone: H2
QHYHTYPFT

SEQ ID NO: 124 - protein, 12 aa, Artificial Sequence
  Synthetic Light chain CDR, clone: E2
QQYYLTPTFTVT

SEQ ID NO: 125 - protein, 9 aa, Artificial Sequence
  Synthetic Light chain CDR, clone: F4
QQTNTFPLT

SEQ ID NO: 126 - protein, 9 aa, Artificial Sequence
  Synthetic Light chain CDR, clone: C5
QQYHTTPYT

SEQ ID NO: 127 - protein, 9 aa, Artificial Sequence
  Synthetic Light chain CDR, clone: E5
QQSFSSPWT

SEQ ID NO: 128 - protein, 9 aa, Artificial Sequence
  Synthetic Light chain CDR, clone: F6
QQSFTTLVT

SEQ ID NO: 129 - protein, 10 aa, Artificial Sequence
  Synthetic Light chain CDR, clone: G5
CQQFNSYPLS

SEQ ID NO: 130 - protein, 13 aa, Artificial Sequence
  Synthetic Light chain CDR, clone: A5
GADHGSGSNLVYV

SEQ ID NO: 131 - protein, 13 aa, Artificial Sequence
  Synthetic Light chain CDR, clone: D6
GADHGSGSDFVYV

SEQ ID NO: 132 - protein, 11 aa, Artificial Sequence
  Synthetic Light chain CDR, clone: E4
AAWDDSLNGPV

SEQ ID NO: 133 - protein, 11 aa, Artificial Sequence
  Synthetic Light chain CDR, clone: F5
AAWDDRLSGPV

SEQ ID NO: 134 - protein, 13 aa, Artificial Sequence
  Synthetic Light chain CDR, clone: G1
ATWDDDLSNPKWV

SEQ ID NO: 135 - protein, 9 aa, Artificial Sequence
  Synthetic Light chain CDR, clone: E3
MQALQTSWT

SEQ ID NO: 136 - protein, 9 aa, Artificial Sequence
  Synthetic Light chain CDR, clone: A2
MQGTHWPYT

SEQ ID NO: 137 - protein, 9 aa, Artificial Sequence
  Synthetic Light chain CDR, clone: D1
MQSRNLPKT

SEQ ID NO: 138 - protein, 8 aa, Artificial Sequence
  Synthetic Light chain CDR, clone: C4
MVWYSAWV

SEQ ID NO: 139 - protein, 10 aa, Artificial Sequence
  Synthetic Light chain CDR, clone: E1
HVLDSSTIVI

SEQ ID NO: 140 - protein, 10 aa, Artificial Sequence
  Synthetic Light chain CDR, clone: A6
HQYNNWPLYT

SEQ ID NO: 141 - protein, 11 aa, Artificial Sequence
  Synthetic Light chain CDR, clone: H1
NSRDSSGYLLL

SEQ ID NO: 142 - protein, 9 aa, Artificial Sequence
  Synthetic Light chain CDR, clone: B2
LLSYSGAGV

SEQ ID NO: 143 - protein, 9 aa, Artificial Sequence
  Synthetic Light chain CDR, clone: C2
LQDYSFPYT

SEQ ID NO: 144 - protein, 9 aa, Artificial Sequence
  Synthetic Light chain CDR, clone: G3
QAWDSSHAV

SEQ ID NO: 145 - protein, 9 aa, Artificial Sequence
  Synthetic Light chain CDR, clone: H3
QSEDSRGPV

SEQ ID NO: 146 - protein, 9 aa, Artificial Sequence
  Synthetic Light chain CDR, clone: D4
VQATHFPVT

SEQ ID NO: 147 - protein, 11 aa, Artificial Sequence
  Synthetic Light chain CDR, clone: C6
CSYTTGSTLYL

SEQ ID NO: 148 - protein, 6 aa, Artificial Sequence
  Synthetic Light chain CDR, clone: B10
AYQSVS

SEQ ID NO: 149 - protein, 6 aa, Artificial Sequence
  Synthetic Light chain CDR, clone: H10
SSQSFS

SEQ ID NO: 150 - protein, 6 aa, Artificial Sequence
  Synthetic Light chain CDR, clone: F10
ASQSMS

SEQ ID NO: 151 - protein, 6 aa, Artificial Sequence
  Synthetic Light chain CDR, clone: B12
ASQPFS

SEQ ID NO: 152 - protein, 7 aa, Artificial Sequence
  Synthetic Light chain CDR, clone: B11
GASSRAS

SEQ ID NO: 153 - protein, 7 aa, Artificial Sequence
  Synthetic Light chain CDR, clone: E7
GASSRAT

SEQ ID NO: 154 - protein, 7 aa, Artificial Sequence
  Synthetic Light chain CDR, clone: E8
GASSRAT

SEQ ID NO: 155 - protein, 7 aa, Artificial Sequence
  Synthetic Light chain CDR, clone: H8
GASSRAT

SEQ ID NO: 156 - protein, 7 aa, Artificial Sequence
  Synthetic Light chain CDR, clone: H12
GASRRAT

SEQ ID NO: 157 - protein, 7 aa, Artificial Sequence
  Synthetic Light chain CDR, clone: F8
VASRRVT

SEQ ID NO: 158 - protein, 7 aa, Artificial Sequence
  Synthetic Light chain CDR, clone: D11
GASSRAT

SEQ ID NO: 159 - protein, 7 aa, Artificial Sequence
  Synthetic Light chain CDR, clone: G8
DASNRAA

SEQ ID NO: 160 - protein, 7 aa, Artificial Sequence
  Synthetic Light chain CDR, clone: H9
RASTRAT

SEQ ID NO: 161 - protein, 6 aa, Artificial Sequence
  Synthetic Light chain CDR, clone: H11
ASQSFS

SEQ ID NO: 162 - protein, 6 aa, Artificial Sequence
  Synthetic Light chain CDR, clone: G12
SSQSIS

SEQ ID NO: 163 - protein, 7 aa, Artificial Sequence
  Synthetic Light chain CDR, clone: E11
RASTRAT

SEQ ID NO: 164 - protein, 7 aa, Artificial Sequence
  Synthetic Light chain CDR, clone: F12
GENNRPS

SEQ ID NO: 165 - protein, 8 aa, Artificial Sequence
  Synthetic Light chain CDR, clone: C8
YDNYQRFS

SEQ ID NO: 166 - protein, 7 aa, Artificial Sequence
  Synthetic Light chain CDR, clone: A8
LASQSFS

SEQ ID NO: 167 - protein, 7 aa, Artificial Sequence
  Synthetic Light chain CDR, clone: B8
DTSNKQS

SEQ ID NO: 168 - protein, 7 aa, Artificial Sequence
  Synthetic Light chain CDR, clone: F7
WASTRES

SEQ ID NO: 169 - protein, 7 aa, Artificial Sequence
  Synthetic Light chain CDR, clone: B7
RDSNRPS

SEQ ID NO: 170 - protein, 7 aa, Artificial Sequence
  Synthetic Light chain CDR, clone: G9
GKDNRPS

SEQ ID NO: 171 - protein, 7 aa, Artificial Sequence
  Synthetic Light chain CDR, clone: A9
DTHNRHS

SEQ ID NO: 172 - protein, 8 aa, Artificial Sequence
  Synthetic Light chain CDR, clone: A11
GIVGSKGD

SEQ ID NO: 173 - protein, 7 aa, Artificial Sequence
  Synthetic Light chain CDR, clone: E12
FDSDRPS

SEQ ID NO: 174 - protein, 7 aa, Artificial Sequence
  Synthetic Light chain CDR, clone: H7
YASQSFS

SEQ ID NO: 175 - protein, 7 aa, Artificial Sequence
  Synthetic Light chain CDR, clone: A10
GNNQRPS

SEQ ID NO: 176 - protein, 7 aa, Artificial Sequence
  Synthetic Light chain CDR, clone: C11
EVSKRFS

SEQ ID NO: 177 - protein, 7 aa, Artificial Sequence
  Synthetic Light chain CDR, clone: D10
DASHLEA

SEQ ID NO: 178 - protein, 7 aa, Artificial Sequence
  Synthetic Light chain CDR, clone: D12
GASSRAA

SEQ ID NO: 179 - protein, 7 aa, Artificial Sequence
  Synthetic Light chain CDR, clone: C7
EVSGRFS

SEQ ID NO: 180 - protein, 7 aa, Artificial Sequence
  Synthetic Light chain CDR, clone: D7
SVSKRDS

SEQ ID NO: 181 - protein, 7 aa, Artificial Sequence
  Synthetic Light chain CDR, clone: C9
EASRLES

SEQ ID NO: 182 - protein, 7 aa, Artificial Sequence
  Synthetic Light chain CDR, clone: C12
GASGLQS

SEQ ID NO: 183 - protein, 7 aa, Artificial Sequence
  Synthetic Light chain CDR, clone: D8
DASNRAT

SEQ ID NO: 184 - protein, 7 aa, Artificial Sequence
  Synthetic Light chain CDR, clone: D9
GASTRAT

SEQ ID NO: 185 - protein, 7 aa, Artificial Sequence
  Synthetic Light chain CDR, clone: G7
KISNRMS

SEQ ID NO: 186 - protein, 7 aa, Artificial Sequence
  Synthetic Light chain CDR, clone: G11
GGSIRAS

SEQ ID NO: 187 - protein, 7 aa, Artificial Sequence
  Synthetic Light chain CDR, clone: F9
AASTLHY

SEQ ID NO: 188 - protein, 7 aa, Artificial Sequence
  Synthetic Light chain CDR, clone: E9
AASRLQS

SEQ ID NO: 189 - protein, 7 aa, Artificial Sequence
  Synthetic Light chain CDR, clone: B1
DDSDRPS

SEQ ID NO: 190 - protein, 7 aa, Artificial Sequence
  Synthetic Light chain CDR, clone: E6
YDNDRPS

SEQ ID NO: 191 - protein, 7 aa, Artificial Sequence
  Synthetic Light chain CDR, clone: F3
YDSDRPS

SEQ ID NO: 192 - protein, 7 aa, Artificial Sequence
  Synthetic Light chain CDR, clone: H4
DDSDRPS

SEQ ID NO: 193 - protein, 7 aa, Artificial Sequence
  Synthetic Light chain CDR, clone: H5
SDRDRPS

SEQ ID NO: 194 - protein, 7 aa, Artificial Sequence
  Synthetic Light chain CDR, clone: B5
DDYGRPS

SEQ ID NO: 195 - protein, 7 aa, Artificial Sequence
  Synthetic Light chain CDR, clone: G6
QDTKRPS

SEQ ID NO: 196 - protein, 7 aa, Artificial Sequence
  Synthetic Light chain CDR, clone: C1
GASSRAT

SEQ ID NO: 197 - protein, 7 aa, Artificial Sequence
  Synthetic Light chain CDR, clone: F1
GASNLEG

SEQ ID NO: 198 - protein, 7 aa, Artificial Sequence
  Synthetic Light chain CDR, clone: A3
GASTLES

SEQ ID NO: 199 - protein, 7 aa, Artificial Sequence
  Synthetic Light chain CDR, clone: B4
EASNLET

SEQ ID NO: 200 - protein, 7 aa, Artificial Sequence
  Synthetic Light chain CDR, clone: B6
AASNRAT

SEQ ID NO: 201 - protein, 7 aa, Artificial Sequence
  Synthetic Light chain CDR, clone: F2
GASNLER

SEQ ID NO: 202 - protein, 7 aa, Artificial Sequence
  Synthetic Light chain CDR, clone: D3
AASYLQT

SEQ ID NO: 203 - protein, 7 aa, Artificial Sequence
  Synthetic Light chain CDR, clone: G2
KVSTLES

SEQ ID NO: 204 - protein, 7 aa, Artificial Sequence
  Synthetic Light chain CDR, clone: A4
EASNLET

SEQ ID NO: 205 - protein, 7 aa, Artificial Sequence
  Synthetic Light chain CDR, clone: G4
GASTRAT

SEQ ID NO: 206 - protein, 7 aa, Artificial Sequence
  Synthetic Light chain CDR, clone: D5
AASTLHY

SEQ ID NO: 207 - protein, 7 aa, Artificial Sequence
  Synthetic Light chain CDR, clone: A1
EASTRAT

SEQ ID NO: 208 - protein, 7 aa, Artificial Sequence
  Synthetic Light chain CDR, clone: H2
QASSLKT

SEQ ID NO: 209 - protein, 7 aa, Artificial Sequence
  Synthetic Light chain CDR, clone: E2
WASTRES

SEQ ID NO: 210 - protein, 7 aa, Artificial Sequence
  Synthetic Light chain CDR, clone: F4
RATNLQS

SEQ ID NO: 211 - protein, 7 aa, Artificial Sequence
  Synthetic Light chain CDR, clone: C5
WASTRES

SEQ ID NO: 212 - protein, 7 aa, Artificial Sequence
  Synthetic Light chain CDR, clone: E5
AASNLQS

SEQ ID NO: 213 - protein, 7 aa, Artificial Sequence
  Synthetic Light chain CDR, clone: F6
SASTLQS

SEQ ID NO: 214 - protein, 7 aa, Artificial Sequence
  Synthetic Light chain CDR, clone: G5
DASTLQT

SEQ ID NO: 215 - protein, 12 aa, Artificial Sequence
  Synthetic Light chain CDR, clone: A5
VGTGGIVGSRGD

SEQ ID NO: 216 - protein, 12 aa, Artificial Sequence
  Synthetic Light chain CDR, clone: D6
VGTGGIVGSRGD

SEQ ID NO: 217 - protein, 7 aa, Artificial Sequence
  Synthetic Light chain CDR, clone: E4
TNNQRPS

SEQ ID NO: 218 - protein, 7 aa, Artificial Sequence
  Synthetic Light chain CDR, clone: F5
TTDRRPS

SEQ ID NO: 219 - protein, 7 aa, Artificial Sequence
  Synthetic Light chain CDR, clone: G1
TTNQRPS

SEQ ID NO: 220 - protein, 7 aa, Artificial Sequence
  Synthetic Light chain CDR, clone: E3
LGSNRAS

SEQ ID NO: 221 - protein, 7 aa, Artificial Sequence
  Synthetic Light chain CDR, clone: A2
QVSTRDS

SEQ ID NO: 222 - protein, 7 aa, Artificial Sequence
  Synthetic Light chain CDR, clone: D1
EASSRFS

SEQ ID NO: 223 - protein, 10 aa, Artificial Sequence
  Synthetic Light chain CDR, clone: C4
RSDSDRHQGS

SEQ ID NO: 224 - protein, 7 aa, Artificial Sequence
  Synthetic Light chain CDR, clone: E1
RDTNRPS

SEQ ID NO: 225 - protein, 7 aa, Artificial Sequence
  Synthetic Light chain CDR, clone: A6
GASTRAT

SEQ ID NO: 226 - protein, 7 aa, Artificial Sequence
  Synthetic Light chain CDR, clone: H1
GKNTRPS

SEQ ID NO: 227 - protein, 7 aa, Artificial Sequence
  Synthetic Light chain CDR, clone: B2
DASNKHS

SEQ ID NO: 228 - protein, 7 aa, Artificial Sequence
  Synthetic Light chain CDR, clone: C2
DSSTLQS

SEQ ID NO: 229 - protein, 7 aa, Artificial Sequence
  Synthetic Light chain CDR, clone: G3
QDTKRPS

SEQ ID NO: 230 - protein, 7 aa, Artificial Sequence
  Synthetic Light chain CDR, clone: H3
KDTERPS

SEQ ID NO: 231 - protein, 7 aa, Artificial Sequence
  Synthetic Light chain CDR, clone: D4
KISNRFS

SEQ ID NO: 232 - protein, 7 aa, Artificial Sequence
  Synthetic Light chain CDR, clone: C6
DVNRRPS

SEQ ID NO: 233 - protein, 11 aa, Artificial Sequence
  Synthetic Light chain CDR, clone: B10
RASQTIGSTLH

SEQ ID NO: 234 - protein, 11 aa, Artificial Sequence
  Synthetic Light chain CDR, clone: H10
RASQSIGSSLH

SEQ ID NO: 235 - protein, 9 aa, Artificial Sequence
  Synthetic Light chain CDR, clone: F10
HQSSSLPWT

SEQ ID NO: 236 - protein, 11 aa, Artificial Sequence
  Synthetic Light chain CDR, clone: B12
RASQSIGIKLH

SEQ ID NO: 237 - protein, 12 aa, Artificial Sequence
  Synthetic Light chain CDR, clone: B11
RASQSVSSNYLA

SEQ ID NO: 238 - protein, 12 aa, Artificial Sequence
  Synthetic Light chain CDR, clone: E7
RASQSVSSSYLA

SEQ ID NO: 239 - protein, 12 aa, Artificial Sequence
  Synthetic Light chain CDR, clone: E8
RASQSVSSSYLA

SEQ ID NO: 240 - protein, 12 aa, Artificial Sequence
  Synthetic Light chain CDR, clone: H8
RASQSVSSNYLA

SEQ ID NO: 241 - protein, 12 aa, Artificial Sequence
  Synthetic Light chain CDR, clone: H12
RASQSVRSSYVA

SEQ ID NO: 242 - protein, 13 aa, Artificial Sequence
  Synthetic Light chain CDR, clone: F8
SGGRSNIGGNAVN

SEQ ID NO: 243 - protein, 12 aa, Artificial Sequence
  Synthetic Light chain CDR, clone: D11
RASQNITSNFFA

SEQ ID NO: 244 - protein, 12 aa, Artificial Sequence
  Synthetic Light chain CDR, clone: G8
RASQSLSGTYLA

SEQ ID NO: 245 - protein, 12 aa, Artificial Sequence
  Synthetic Light chain CDR, clone: H9
RASEDIYNNYLA

SEQ ID NO: 246 - protein, 11 aa, Artificial Sequence
  Synthetic Light chain CDR, clone: H11
RASQSIGSSLH

SEQ ID NO: 247 - protein, 11 aa, Artificial Sequence
  Synthetic Light chain CDR, clone: G12
RASESIGTALH

SEQ ID NO: 248 - protein, 12 aa, Artificial Sequence
  Synthetic Light chain CDR, clone: E11
RTSQILHSQYLA

SEQ ID NO: 249 - protein, 11 aa, Artificial Sequence
  Synthetic Light chain CDR, clone: F12
QGDTLRTCYAS

SEQ ID NO: 250 - protein, 13 aa, Artificial Sequence
  Synthetic Light chain CDR, clone: C8
SGSTSNIGKNFVS

SEQ ID NO: 251 - protein, 11 aa, Artificial Sequence
  Synthetic Light chain CDR, clone: A8
RASRYIGSNLH

SEQ ID NO: 252 - protein, 14 aa, Artificial Sequence
  Synthetic Light chain CDR, clone: B8
GSSTGAVTSGHSPF

SEQ ID NO: 253 - protein, 17 aa, Artificial Sequence
  Synthetic Light chain CDR, clone: F7
  misc_feature (4)..(4): Xaa can be any naturally occurring amino acid
KSSXSLLYRSNNKNYLA

SEQ ID NO: 254 - protein, 11 aa, Artificial Sequence
  Synthetic Light chain CDR, clone: B7
GGANIANKNVH

SEQ ID NO: 255 - protein, 11 aa, Artificial Sequence
  Synthetic Light chain CDR, clone: G9
QGDSLRTYYAS

SEQ ID NO: 256 - protein, 14 aa, Artificial Sequence
  Synthetic Light chain CDR, clone: A9
GSSTGAVTSGHYPY

SEQ ID NO: 257 - protein, 12 aa, Artificial Sequence
  Synthetic Light chain CDR, clone: A11
TLSSGYSNYKVD

SEQ ID NO: 258 - protein, 11 aa, Artificial Sequence
  Synthetic Light chain CDR, clone: E12
GGNNIGSKSVH

SEQ ID NO: 259 - protein, 11 aa, Artificial Sequence
  Synthetic Light chain CDR, clone: H7
RASQNIGNSLH

SEQ ID NO: 260 - protein, 13 aa, Artificial Sequence
  Synthetic Light chain CDR, clone: A10
TRCTGNIASHFVQ

SEQ ID NO: 261 - protein, 17 aa, Artificial Sequence
  Synthetic Light chain CDR, clone: C11
KSSQSLLNSDDGKTYLY

SEQ ID NO: 262 - protein, 11 aa, Artificial Sequence
  Synthetic Light chain CDR, clone: D10
QASHDISNYLN

SEQ ID NO: 263 - protein, 12 aa, Artificial Sequence
  Synthetic Light chain CDR, clone: D12
RASQSVSRTYLA

SEQ ID NO: 264 - protein, 16 aa, Artificial Sequence
  Synthetic Light chain CDR, clone: C7
KSSQSLLHSDGKTHLF

SEQ ID NO: 265 - protein, 16 aa, Artificial Sequence
  Synthetic Light chain CDR, clone: D7
RSSHSLVHSDGNIYLN

SEQ ID NO: 266 - protein, 11 aa, Artificial Sequence
  Synthetic Light chain CDR, clone: C9
RASQSISSWLA

SEQ ID NO: 267 - protein, 11 aa, Artificial Sequence
  Synthetic Light chain CDR, clone: C12
RTSQGIRNYLS

SEQ ID NO: 268 - protein, 12 aa, Artificial Sequence
  Synthetic Light chain CDR, clone: D8
RASQSVTSNYLA

SEQ ID NO: 269 - protein, 11 aa, Artificial Sequence
  Synthetic Light chain CDR, clone: D9
RASQSVSSKLA

SEQ ID NO: 270 - protein, 16 aa, Artificial Sequence
  Synthetic Light chain CDR, clone: G7
RSSESPVHSDGNIYLS

SEQ ID NO: 271 - protein, 12 aa, Artificial Sequence
  Synthetic Light chain CDR, clone: G11
RASQSVSSRNLA

SEQ ID NO: 272 - protein, 11 aa, Artificial Sequence
  Synthetic Light chain CDR, clone: F9
RASDNIGNYLN

SEQ ID NO: 273 - protein, 11 aa, Artificial Sequence
  Synthetic Light chain CDR, clone: E9
RASESISNYLN

SEQ ID NO: 274 - protein, 11 aa, Artificial Sequence
  Synthetic Light chain CDR, clone: B1
GGNNIGYDSVH

SEQ ID NO: 275 - protein, 10 aa, Artificial Sequence
  Synthetic Light chain CDR, clone: E6
GGNNIGATTV

SEQ ID NO: 276 - protein, 11 aa, Artificial Sequence
  Synthetic Light chain CDR, clone: F3
GGNNIGSKSVH

SEQ ID NO: 277 - protein, 11 aa, Artificial Sequence
  Synthetic Light chain CDR, clone: H4
GGNNIVSKGVH

SEQ ID NO: 278 - protein, 11 aa, Artificial Sequence
  Synthetic Light chain CDR, clone: H5
GGNNLGSKIVH

SEQ ID NO: 279 - protein, 11 aa, Artificial Sequence
  Synthetic Light chain CDR, clone: B5
AGNNIGGKSVQ

SEQ ID NO: 280 - protein, 11 aa, Artificial Sequence
  Synthetic Light chain CDR, clone: G6
SGDNLGHTNAC

SEQ ID NO: 281 - protein, 12 aa, Artificial Sequence
  Synthetic Light chain CDR, clone: C1
TASQSVSSTYLT

SEQ ID NO: 282 - protein, 11 aa, Artificial Sequence
  Synthetic Light chain CDR, clone: F1
RASQNIDYDLA

SEQ ID NO: 283 - protein, 11 aa, Artificial Sequence
  Synthetic Light chain CDR, clone: A3
QASQVIDKYVN

SEQ ID NO: 284 - protein, 11 aa, Artificial Sequence
  Synthetic Light chain CDR, clone: B4
QASQDIFHYLN

SEQ ID NO: 285 - protein, 12 aa, Artificial Sequence
  Synthetic Light chain CDR, clone: B6
RASQSFGSNYLA

SEQ ID NO: 286 - protein, 11 aa, Artificial Sequence
  Synthetic Light chain CDR, clone: F2
QASQFIHIYLN

SEQ ID NO: 287 - protein, 11 aa, Artificial Sequence
  Synthetic Light chain CDR, clone: D3
RASQDVGIYVA

SEQ ID NO: 288 - protein, 11 aa, Artificial Sequence
  Synthetic Light chain CDR, clone: G2
RASQDINTWLA

SEQ ID NO: 289 - protein, 11 aa, Artificial Sequence
  Synthetic Light chain CDR, clone: A4
QASQDISNWLN

SEQ ID NO: 290 - protein, 11 aa, Artificial Sequence
  Synthetic Light chain CDR, clone: G4
RVSQNVFSDLA

SEQ ID NO: 291 - protein, 11 aa, Artificial Sequence
  Synthetic Light chain CDR, clone: D5
RASDNIGNYLN

SEQ ID NO: 292 - protein, 11 aa, Artificial Sequence
  Synthetic Light chain CDR, clone: A1
RASQSVSSFLA

SEQ ID NO: 293 - protein, 11 aa, Artificial Sequence
  Synthetic Light chain CDR, clone: H2
RATESISIWLA

SEQ ID NO: 294 - protein, 17 aa, Artificial Sequence
  Synthetic Light chain CDR, clone: E2
KSSQSVLYSSNNKNYLA

SEQ ID NO: 295 - protein, 11 aa, Artificial Sequence
  Synthetic Light chain CDR, clone: F4
RASQDISSWLA

SEQ ID NO: 296 - protein, 17 aa, Artificial Sequence
  Synthetic Light chain CDR, clone: C5
KSSQSVLYSSNNRNYLA

SEQ ID NO: 297 - protein, 11 aa, Artificial Sequence
  Synthetic Light chain CDR, clone: E5
RASQTFTSHLN

SEQ ID NO: 298 - protein, 11 aa, Artificial Sequence
  Synthetic Light chain CDR, clone: F6
RASQSVNVYLN

SEQ ID NO: 299 - protein, 11 aa, Artificial Sequence
  Synthetic Light chain CDR, clone: G5
RASQDISSSLA

SEQ ID NO: 300 - protein, 12 aa, Artificial Sequence
  Synthetic Light chain CDR, clone: A5
TVSSGYRSYEVD

SEQ ID NO: 301 - protein, 12 aa, Artificial Sequence
  Synthetic Light chain CDR, clone: D6
TLSSDYSSYNVD

SEQ ID NO: 302 - protein, 13 aa, Artificial Sequence
  Synthetic Light chain CDR, clone: E4
SGSSTNIGSNAVN

SEQ ID NO: 303 - protein, 13 aa, Artificial Sequence
  Synthetic Light chain CDR, clone: F5
SGGGSNIGSNFGY

SEQ ID NO: 304 - protein, 13 aa, Artificial Sequence
  Synthetic Light chain CDR, clone: G1
SGSSSNIGSNSVD

SEQ ID NO: 305 - protein, 16 aa, Artificial Sequence
  Synthetic Light chain CDR, clone: E3
RSSQSLLHSNGYNFLD

SEQ ID NO: 306 - protein, 13 aa, Artificial Sequence
  Synthetic Light chain CDR, clone: A2
CDDTVSTLPARHP

SEQ ID NO: 307 - protein, 16 aa, Artificial Sequence
  Synthetic Light chain CDR, clone: D1
KSSQSLVHRDGKTYLY

SEQ ID NO: 308 - protein, 14 aa, Artificial Sequence
  Synthetic Light chain CDR, clone: C4
TLSSGFNVVSYNIY

SEQ ID NO: 309 - protein, 11 aa, Artificial Sequence
  Synthetic Light chain CDR, clone: E1
AGNNIGTYYVH

SEQ ID NO: 310 - protein, 11 aa, Artificial Sequence
  Synthetic Light chain CDR, clone: A6
RASQSVSSNLA

SEQ ID NO: 311 - protein, 11 aa, Artificial Sequence
  Synthetic Light chain CDR, clone: H1
QGDSLRTYYAS

SEQ ID NO: 312 - protein, 14 aa, Artificial Sequence
  Synthetic Light chain CDR, clone: B2
GSSTGAVTSGHYPY

SEQ ID NO: 313 - protein, 11 aa, Artificial Sequence
  Synthetic Light chain CDR, clone: C2
RPSQDIGTDLG

SEQ ID NO: 314 - protein, 11 aa, Artificial Sequence
  Synthetic Light chain CDR, clone: G3
SGDELKYKYTC

SEQ ID NO: 315 - protein, 11 aa, Artificial Sequence
  Synthetic Light chain CDR, clone: H3
SGSTFPKLYSF

SEQ ID NO: 316 - protein, 16 aa, Artificial Sequence
  Synthetic Light chain CDR, clone: D4
RSSESVVHDDGNTYLS

SEQ ID NO: 317 - protein, 14 aa, Artificial Sequence
  Synthetic Light chain CDR, clone: C6
TGTSDDVGRYDYVS

SEQ ID NO: 318 - protein, 116 aa, Artificial Sequence
  Synthetic Heavy chain, clone:  A4 XB1511
QVQLVQSGAEVKKPGSSVKVSCKASGGTFSSYAISWVRQAPGQGLEWMGGIIPIFGTANYAQKFQGRVTITADESTSTAYMELSSLRSEDTAVYYCAIHGGDRSYWGQGTLVTVSS

SEQ ID NO: 319 - protein, 116 aa, Artificial Sequence
  Synthetic Heavy chain, clone:  B4
QVQLVQSGAEVKKPGASVKVSCKASGYTFTSYAISWVRQAPGQGLEWMGGIIPIFGTANYAQKFQGRVTITADESTSTAYMELSSLRSEDTAVYYCAIHGGDRSYWGQGTLVTVSS

SEQ ID NO: 320 - protein, 116 aa, Artificial Sequence
  Synthetic Heavy chain, clone:  G2
QVQLVQSGAEVKKPGASVKVSCKASGYTFTGYAISWVRQAPGQGLEWMGGIIPIFGTANYAQKFQGRVTITADESTSTAYMELSSLRSKDTAVYYCAIHGGDRSYWGQGTLVTVSS

SEQ ID NO: 321 - protein, 116 aa, Artificial Sequence
  Synthetic Heavy chain, clone:  XB2202
QVQLVQSGAEVKKPGSSVRVSCKASGGTFSRHAISWVRQAPGQGLEWIGGILPILKTPNYAQRFQGRVTINADESTSTVYMEMSSLRSEDTAVYYCATHGGDRSYWGQGTLVTVSS

SEQ ID NO: 322 - protein, 116 aa, Artificial Sequence
  Synthetic Heavy chain, clone:  C4
QMQLVQSGAEVKKPGSSVRVSCKASGGTFSRHAISWVRQAPGQGLEWIGGILPILKTPNYAQRFQGRVTINADESTSTVYMEMSGLRSEDTAVYYCATHGGDRSYWGQGTLVTVSS

SEQ ID NO: 323 - protein, 116 aa, Artificial Sequence
  Synthetic Heavy chain, clone:  B12
QMQLVQSGAEVKKPGSSVRVSCKASGGTFSRHAISWVRQAPGQGLEWIGGILPILKTPNYAQRFQGRVTINADESTSTVYMEMSSLRSENTAVYYCATHGGDRSYWGQGTLVTVSS

SEQ ID NO: 324 - protein, 116 aa, Artificial Sequence
  Synthetic Heavy chain, clone:  D07
QMQLVQSGAEVKKPGSSVRVSCKASGGTFSRHAISWVRQAPGQGLEWIGGILPILKTPNYAQRFQGRVTINADESTSTVYMEMSSLRSDDTAVYYCATHGGDRSYWGQGTLVTVSS

SEQ ID NO: 325 - protein, 116 aa, Artificial Sequence
  Synthetic Heavy chain, clone:  C05
QMQLVQSGAEVKKPGSSVRVSCKASGGTFSRHAISWVRQAPGQGLEWIGGVLPILKTPNYAQRFQGRVTINADESTSTVYMELSSLRSEDTAVYYCATHGGDRSYWGQGTLVTVSS

SEQ ID NO: 326 - protein, 116 aa, Artificial Sequence
  Synthetic Heavy chain, clone:  E05
QVQLVQSGPKVKKPGSSVRVSCKASGGTFSRHAISWVRQAPGQGLEWIGGILPILKTPNYAQRFQGRVTINADESTSTVYMEMSSLRSEDTAVYYCATHGGDRSYWGQGTLVTVSS

SEQ ID NO: 327 - protein, 116 aa, Artificial Sequence
  Synthetic Heavy chain, clone:  E2
QMQLVQSGAEVKKPGASVKISCKTSGYTFTDYYIQWVRQAPGQGLEWVGWINPNSGNTGYAQKFQGRVTMTRDTSISTAYMELSSLRSEDTAVYYCATHGGDYSYWGQGTLVTVSS

SEQ ID NO: 328 - protein, 116 aa, Artificial Sequence
  Synthetic Heavy chain, clone:  A3
QVQLVQSGAEVKKPGASVRVSCKASGYTFSDYYIQWVRQAPGQGLEWMGWINPNSGGTYFAQKFQGRVTMTRDTSISTAYMELSSLTSDDTAVYYCATHGGDRGYWGQGTLVTVSS

SEQ ID NO: 329 - protein, 116 aa, Artificial Sequence
  Synthetic Heavy chain, clone:  C3
QMQLVQSGAEVKKPGASVKVSCKASGYTFTDYYIQWVRQAPGQGLEWIGGILPILKTPNYAQRFQGRVTINADESTSTVYMEMSSLRSEDTAVYYCATHGGDRSYWGQGTLVTVSS

SEQ ID NO: 330 - protein, 116 aa, Artificial Sequence
  Synthetic Heavy chain, clone:  F10
QMQLVQSGAEVKKPGASVKVSCKASGYTFTDYYIQWVRQAPGQGLEWMGWINPDSGGTYFAQKFQGRVAMTRDTSINTAYMELSSLRSDDTAVYYCATHGGDRSYWGQGTLVTVSS

SEQ ID NO: 331 - protein, 116 aa, Artificial Sequence
  Synthetic Heavy chain, clone:  C12
QVQLVQSGAEVKKPGASVKVSCKASGYTFTDYYIQWVRQAPGEGLEWMGWMNPDSGGTIYAQKFQGRVTMTRDTSISTAYMELSRLRPDDTAVYYCATHGGDRSYWGQGTLVTVSS

SEQ ID NO: 332 - protein, 116 aa, Artificial Sequence
  Synthetic Heavy chain, clone:  H2
QMQLVQSGAEVKNPGASVKVSCKASGYPFSAYYIQWVRQAPGQGLEWMGWLNPNSGDTHSAQKFQGRVTMTRDTSISTAYMELSGLTSDDTAVYYCATHGGDRSYWGQGTLVTVSS

SEQ ID NO: 333 - protein, 116 aa, Artificial Sequence
  Synthetic Heavy chain, clone:  F11
QMQLVQSGAEVKNPGASVKVSCKASGYPFSAYYIQWVRQAPGQGLEWMGWLNPNSGDTHSAQKFQGRVTMTRDTSISTAYMELSGPTSDDTAVYYCATHGGDRSYWGQGTLVTVSS

SEQ ID NO: 334 - protein, 116 aa, Artificial Sequence
  Synthetic Heavy chain, clone:  B1
QMQLVQSGAEVRKPGASVKVSCKASGYSFSDYYIHWVRQAPGQGLEWIGWINPNNGNTTYAQKFQGRVTMIRDTSISTAYMELSELRSDDTAVYYCATHGGDRSYWGQGTLVTVSS

SEQ ID NO: 335 - protein, 116 aa, Artificial Sequence
  Synthetic Heavy chain, clone:  E11
QVQLVQSGAEVEKPGASVKVSCKASGYTFTDYYIHWVRQAPGQGLEWMRGIIPIFGTANYAQKFQGRVTITADESTSTAYMELSSLRSEDTAVYYCATHGGDRSYWGQGTLVTVSS

SEQ ID NO: 336 - protein, 116 aa, Artificial Sequence
  Synthetic Heavy chain, clone:  H1
EVQLLESGAEVKQPGASVKVSCKTSGYTFTDYHLHWVRQAPGQGLEWMGWINPNSGGTNSAPKFQGRVTMTRDTSISTAYMELSGLTSDDTAVYYCATHGGDRSYWGQGTLVTVSS

SEQ ID NO: 337 - protein, 116 aa, Artificial Sequence
  Synthetic Heavy chain, clone:  E6
QMQLVQSGAEVKRPGASVKVPCKASGYTFTDYYLHWVRQAPGQGLKWMGWINPNSGGTNYAQKFQGRVTMTRDTSISTAYMELSRLRSEDTAVYYCATHGGDRSYWGQGTLVTVSS

SEQ ID NO: 338 - protein, 116 aa, Artificial Sequence
  Synthetic Heavy chain, clone:  A1
QVQLVQSGPEVKKPGTSVKVSCKASGFTFTSSAVQWVRQARGQRLEWIGWIVVGSGNTNYAQKFQERVTITRDMSTSTAYMELSSLRSEDTAVYYCATHGGDRSYWGQGTLVTVSS

SEQ ID NO: 339 - protein, 116 aa, Artificial Sequence
  Synthetic Heavy chain, clone:  H7
QVQLVQSGPEVKKPGTSVKVSCKASGFTFTSSAMQWVRQARGQRLEWIGWIVVGSGNTNYAQKFQERVTITRDMSTSTAYMELSSLRSEDTAVYYCATHGGDRSYWGQGTLVTVSS

SEQ ID NO: 340 - protein, 116 aa, Artificial Sequence
  Synthetic Heavy chain, clone:  G04
QVQLVQSGAEVKKPGASVKVSCKASGFTFTSYAISWVRQARGQRLEWIGWIVVGSGNTNYAQKFQERVTITRDMSTSTAYMELSSLRSEDTAVYYCATHGGDRSYWGQGTLVTVSS

SEQ ID NO: 341 - protein, 116 aa, Artificial Sequence
  Synthetic Heavy chain, clone:  B2
QVQLVQSGAEVKKPGASVKVSCKASGYSFTNYQVQWVRQAPGQGLEWLGVINTGVGSTNYAQKFQGRVTMTRDTATSTVYMELSSLRSEDTAVYYCATHGGDRSYWGQGTLVTVSS

SEQ ID NO: 342 - protein, 116 aa, Artificial Sequence
  Synthetic Heavy chain, clone:  A7
QVQLVQSGAEVKKPGASVKVSCKASGYSFTNYPVQWVRQAPGQGLEWLGVINTGVGSTNYAQKFQGRVTMTRDTATSIVYMELSSLRSEDTAVYYCATHGGDRSYWGQGTLVTVSS

SEQ ID NO: 343 - protein, 116 aa, Artificial Sequence
  Synthetic Heavy chain, clone:  H3
QVQLVQSGAEVKKPGASVKVSCRASGYTFTNSFMQWVRQVPGQRLEWVGLSNPSGDYTVYAPKFQGRVTMTTDTATSTFYMELFSLRSDDTAVYYCATHGGDRSYWGQGTLVTVSS

SEQ ID NO: 344 - protein, 116 aa, Artificial Sequence
  Synthetic Heavy chain, clone:  B4
QVQLVQSGAEVKKPGASVKVSCRASGYTFTNSFMQWVRQVPGQRLEWVGLSNPSGDYTVYAPKLQGRVTMTTDTATGTFYMELFSLRSDDTAVYYCATHGGDRSYWGQGTLVTVSS

SEQ ID NO: 345 - protein, 116 aa, Artificial Sequence
  Synthetic Heavy chain, clone:  H05
EVQLVQSGGGVVQPGGSLRLSCAASGFTFRSYGMHWVRQAPGKGLEWVAFILFDGNNKYYADSVKGRFTISSDNSKNTLYLQMNSLRAEDTAVYYCATHGGDRSYWGQGTLVTVSS

SEQ ID NO: 346 - protein, 116 aa, Artificial Sequence
  Synthetic Heavy chain, clone:  D06
QVQLVQSGGGVVQPGRSLRLSCAASGFTFSSYGMHWVRQAPGKGLEWVAVISYDGSNKYYADSVKGRFTISRDNSKNTLYLQMNSLRAEDTAVYYCAKHGGDRSYWGQGTLVTVSS

SEQ ID NO: 347 - protein, 116 aa, Artificial Sequence
  Synthetic Heavy chain, clone:  F3
QVQLVQSGAEVKKPGASVKVSCKASGYTFISHGMSWVRQAPGQGLEWMGWISADNGNTNYAQKFQERVTITRDMSTSTAYMELSSLRSEDTAVYYCATHGGDRSYWGQGTLVTVSS

SEQ ID NO: 348 - protein, 116 aa, Artificial Sequence
  Synthetic Heavy chain, clone:  A12
QVQLVQSGAEVKKPGASVKVSCKASGYTFISHGMSWVRQAPGQGLEWMGWISADNGNTKYAQKFQDRVTLTTDTSTSTAYLELRSLRSDDTAVYYCATHGGDRSYWGQGTLVTVSS

SEQ ID NO: 349 - protein, 116 aa, Artificial Sequence
  Synthetic Heavy chain, clone:  G3
QVQLVQSGAEVKKPGASVKVSCKVSGYTLTELSMHWVRQAPGKGLEWMGGFDPEDGETIYAQKFQGRVTMTRDTSISTAYMELSRLRSDDTAVYYCATHGGDRSYWGQGTLVTVSS

SEQ ID NO: 350 - protein, 116 aa, Artificial Sequence
  Synthetic Heavy chain, clone:  F05
QVQLVQSGAEVKRPGASVKVSCKASGYTLTELSMHWVRQAPGKGLEWMGGFDPEDGETIYAQKFQGRVTMTEDTSTDTAYMELSSLRSEDTAVYYCATHGGDRSYWGQGTLVTVSS

SEQ ID NO: 351 - protein, 116 aa, Artificial Sequence
  Synthetic Heavy chain, clone:  H12
QVQLVQSGAEVKKPGASVKVSCKASGYTFTDNYVHWVRQAPGQGLEWMGGIIPIFGTANYAQKFQGRVTITADESTSTAYMELSSLRSEDTAVYYCATHGGDRSYWGQGTLVTVSS

SEQ ID NO: 352 - protein, 116 aa, Artificial Sequence
  Synthetic Heavy chain, clone:  G12
QVQLVQSGAEVKKPGSSVKVSCKASGGAFNAYPISWVRQAPGQGLEWMGGIIPVSGTPNYAQKFQGRVTITADKSTYTAYMELSSLRSEDTAVYYCATHGGDRSYWGQGTLVTVSS

SEQ ID NO: 353 - protein, 116 aa, Artificial Sequence
  Synthetic Heavy chain, clone:  C06
QMQLVQSGAEVKKPGASVKVSCMASGYTFTGHYIHWVRQAPGQGLEWMGGIIPIFGTANYAQKFQGRVTITADESTSTAYTELSSLRSEDTAVYYCATHGGDRSYWGQGTLVTVSS

SEQ ID NO: 354 - protein, 116 aa, Artificial Sequence
  Synthetic Heavy chain, clone:  C11
QVQLVQSGAAVKKPGASVKVSRKASGYTFTNDYIHWVRQAPGQGLEWMGGIIPIFGTANYAQKFQGRVTITADESTSTAYMELSSLRSEDTAVYYCATHGGDRSYWGQGTLVTVSS

SEQ ID NO: 355 - protein, 116 aa, Artificial Sequence
  Synthetic Heavy chain, clone:  F08
QVQLVQSGAEVKKPGASVKVSCKASGYTFTSSYIHWVRQAPGQGLEWMGGIIPIFGTANYAQKFQGRVTITADKSTSTAYMELSSLRSEDTAMYYCATHGGDRSYWGQGTLVTVSS

SEQ ID NO: 356 - protein, 116 aa, Artificial Sequence
  Synthetic Heavy chain, clone:  E9
QVQLVESGAEVRKPGESLQISCKASGYRFTNYWIGWVRQMPGKGLEWMGITYPADSTTVYSPSFQGQVTISADKSISTVFLQWSSLRSEDTAVYYCATHGGDRSYWGQGTLVTVSS

SEQ ID NO: 357 - protein, 116 aa, Artificial Sequence
  Synthetic Heavy chain, clone:  E11
QVQLVESGGGVVQPGRSLRLSCAASGFTFSSYWMHWVRQAPGKGLVWVSRINNDGSSTSYADSVKGRFTISRDTAKNTLYLQMNSLRAEDTAVYYCATHGGDRSYWGQGTLVTVSS

SEQ ID NO: 358 - protein, 116 aa, Artificial Sequence
  Synthetic Heavy chain, clone:  H11
QVQLLESGAEVKNPGASVKVSCKASGYPFSAYYIQWVRQAPGQGLEWMGWLNPNSGDTHSAQKFQGRVTMTRDTSISTAYMELSGLTSDDTAVYYCATHGGDRSYWGQGTLVTVSS

SEQ ID NO: 359 - protein, 116 aa, Artificial Sequence
  Synthetic Heavy chain, clone:  C08
EVQLLESEGGLVQPGGSLRLSCTASGFSFNAFWMHWVRQAPGKGLEWVSRISIDGTTTTYADSVQGRFTISRDNARNTLYLQMNSLRAEDAAVYYCATHGGDRSYWSQGTLVTVSS

SEQ ID NO: 360 - protein, 116 aa, Artificial Sequence
  Synthetic Heavy chain, clone:  XB2708
QVQLVQSGGGVVQPGGSLRLSCAASGFTSRSYGMHWVRQAPGKGLEWVAFILFDGNNKYYADSVKGRFTISSDNSKNTLYLQMNSLRAEDTAVYYCATHGGDRSYWGQGTLVTVSS

SEQ ID NO: 361 - protein, 116 aa, Artificial Sequence
  Synthetic Heavy chain, clone:  D03
QVQLVQSGGGLVQPGGSLRLSCVASGFTFGNDWMHWVRQAPGKGLVWVSRINADGTSTAYAESVKGRFTVSRDNAKNTLYLQMNGLRAEDTAVYYCATHGGDRSYWGQGTLVTVSS

SEQ ID NO: 362 - protein, 115 aa, Artificial Sequence
  Synthetic Heavy chain, clone:  A10
QVQLVQSGGGLVQPGRSLRLSCAASGFTFDDYAMNWVRQAPGKGLEWVSLIYSDGSTYYADSVKGRFTISRDNSKKTLYLQMNNLRVEDTAVYYCATHGGDRSYWGQGTLVTVSS

SEQ ID NO: 363 - protein, 116 aa, Artificial Sequence
  Synthetic Heavy chain, clone:  C09
QVQLVQSGGALVQPGGSLRLSCAASGFTLSNNAMSWVRQAPGKRLEWVSAIDGSGGTTYYAGSVKGRFTISSDNSKNTVFLQMNSLRAEDTAVYYCATHGGDRSYWGQGTLVTVSS

SEQ ID NO: 364 - protein, 116 aa, Artificial Sequence
  Synthetic Heavy chain, clone:  A06
QVQLVQSGGGLVQPGGSLRLSCAASGFTFSGHWMHWVRQVPGKGLVWVSHISNDGSITRYADSVKGRFTVARDNAKNTMYLQMNSLRAEDTAVYYCATHGGDRSYWGQGTLVTVSS

SEQ ID NO: 365 - protein, 116 aa, Artificial Sequence
  Synthetic Heavy chain, clone:  C05
QVQLVQSGGGLVKPGGSLRLSCAASGFIFSSNWMHWVRQVPGKGLEWVSRIKTDGSSTSYADSVKGRFTISRDNAKNTLYLQMNSLRAEDTAVYYCATHGGDRSYWGQGTLVTVSS

SEQ ID NO: 366 - protein, 116 aa, Artificial Sequence
  Synthetic Heavy chain, clone:  H01
QVQLVQSGGGLVQPGGSLRLSCAASGFTLSSDWMHWVRQAPGKGLVWVSRISSDGSTTAYADSVRGRFTISRDNAKNTLYLQMNSLRAEDTAVYYCATHGGDRSYWGQGTLVTVSS

SEQ ID NO: 367 - protein, 116 aa, Artificial Sequence
  Synthetic Heavy chain, clone:  G04
QVQLVQSGGGLVQPGGSLRLSCAASGFTLSSDWMHWVRQAPGKGLVWVSRISSDGSTTAYADSVRGRFTISRDNTKNTLYLQMNSLRAEDTAVYYCATHGGDRSYWGQGTLVTVSS

SEQ ID NO: 368 - protein, 116 aa, Artificial Sequence
  Synthetic Heavy chain, clone:  G07
QVQLVQSGGGLVQPGGSLRLSCAASGFTFSSDWMHWVRQAPGEGLVWVSRISSDGSSTAYADSVKGRFTISRDNAKNTVSLQMNSLRAEDTAVYYCATHGGDRSYWGQGTLVTVSS

SEQ ID NO: 369 - protein, 107 aa, Artificial Sequence
  Synthetic Light chain, clone:  B10
QSVLTQSPDLQSVTPREKLTITCRASQTIGSTLHWYQQKPGQSPRLVIKYAYQSVSGVPSRFSGSGSGTEFTLTINGLEAEDAATYYCHQSSSLPWTFGQGTKLTVL

SEQ ID NO: 370 - protein, 107 aa, Artificial Sequence
  Synthetic Light chain, clone:  H10
QSVLTQSPDFQSVSPKDKVTITCRASQSIGSSLHWYQQKPGQSPKLLIKYSSQSFSGVPSRFSGSASGTEFTLTITGLEAEDAATYYCHQSSSLPHTFGQGTKVTVL

SEQ ID NO: 371 - protein, 107 aa, Artificial Sequence
  Synthetic Light chain, clone:  F10
QSVLTQSPEFQSVTPKEKVTITCRASQSIGSGLHWYQQKPHQSPKLLIRYASQSMSGVPSRFSGSGSGTDFTLTISRLEVEDAAMYYCHQSSSLPWTFGQGTKVTVL

SEQ ID NO: 372 - protein, 107 aa, Artificial Sequence
  Synthetic Light chain, clone:  B12
QSVLTQSPDFQSVTPKQNVTFTCRASQSIGIKLHWYQQKPDQSPKVLIKYASQPFSGVPSRFSGRGSGTDFTLTINSLEAEDAATYYCHQTSSLPLTFGGGTKVTVL

SEQ ID NO: 373 - protein, 108 aa, Artificial Sequence
  Synthetic Light chain, clone:  B11
QSVLTQSPGTLSLSPGERATLSCRASQSVSSNYLAWYQQKPGQAPRLLIYGASSRASGIPVRVSGSGSGTDFTLTISRLEPEDFAVYYCQQYGSSPWTFGQGTKLTVL

SEQ ID NO: 374 - protein, 108 aa, Artificial Sequence
  Synthetic Light chain, clone:  E7
QSVLTQSPGTLSLSPGERATLSCRASQSVSSSYLAWYQQKPGQAPRLLIYGASSRATGIPDRFSGSGSGTDFTLTISRLEPEDFAVYYCQQYGSSPQTFGQGTKLTVL

SEQ ID NO: 375 - protein, 109 aa, Artificial Sequence
  Synthetic Light chain, clone:  E8
QSVLTQSPGTLSLSPGERATLSCRASQSVSSSYLAWYQQKPGQAPRLLIYGASSRATGIPDRFSGSGSGTDFTLTISRLEPEDFAVYYCQQYGSSPPYTFGQGTKLTVL

SEQ ID NO: 376 - protein, 108 aa, Artificial Sequence
  Synthetic Light chain, clone:  H8
QSVLTQSPGTLSLSPGERATLSCRASQSVSSNYLAWYLQKPGQAPRLLISGASSRATGIPDRFSGSGSGTDFTLTISRLEPEDFAVYYCQQYAGSPFTFGPGTKLTVL

SEQ ID NO: 377 - protein, 108 aa, Artificial Sequence
  Synthetic Light chain, clone:  H12
QSVLTQSPGTLSLSPGERATLSCRASQSVRSSYVAWYQQKPGQAPRLLISGASRRATGIPDRFTGSGSGTDFTLTISRLEPEDFAVYHCQQFGSSPWTFGQGTKLTVL

SEQ ID NO: 378 - protein, 108 aa, Artificial Sequence
  Synthetic Light chain, clone:  F8
QSVLTQPPSASGTPGQRVTISCSGGRSNIGGNAVNWYQQKPGQAPRLLIHVASRRVTGIPDRFSGSGSGTDFTLTISRLEPEDFAIYYCQQYGSSPLTFGGGTKLTVL

SEQ ID NO: 379 - protein, 108 aa, Artificial Sequence
  Synthetic Light chain, clone:  D11
QSVLTQSPGTLSLSPGERATLSCRASQNITSNFFAWYQQKPGQAPRLLIYGASSRATGIPDRISGSGSGTDFTLTISRLEPEDFALYYCQQYGASPRTFGQGTQLTVL

SEQ ID NO: 380 - protein, 108 aa, Artificial Sequence
  Synthetic Light chain, clone:  G8
QSVLTQSPGTLSLSPGDRATLSCRASQSLSGTYLAWYQQKPGQAPRLLIYDASNRAAGIPKRFSGSGSRTDFTLTISRVDPADSAVYYCQQYGSALLTFGGGTKVTVL

SEQ ID NO: 381 - protein, 107 aa, Artificial Sequence
  Synthetic Light chain, clone:  H9
QSVLTQSPGTLSLSPGESATLSCRASEDIYNNYLAWYQHKRGQPPRLLIFRASTRATGIPTRFSGSGSGRDFVLTINRLEPEDFAVYYCQQYGNSWTFGQGTKLTVL

SEQ ID NO: 382 - protein, 107 aa, Artificial Sequence
  Synthetic Light chain, clone:  H11
QSVLTQSPDFQSVTPKEKVTITCRASQSIGSSLHWYQQKPDQSPKLLITFASQSFSGVPSRFSGSGSGTDFTLTINSLEAEDAATYYCHQSRNLPFTFGPGTKLTVL

SEQ ID NO: 383 - protein, 107 aa, Artificial Sequence
  Synthetic Light chain, clone:  G12
QSVLTQSPDFQSVTPKEEVTITCRASESIGTALHWYQQKPDQSPKLLIKYSSQSISGVPSRFVGRGSETEFTLTINSLEAENAATYYCHQSRSFPLTFGQGTQLTVL

SEQ ID NO: 384 - protein, 107 aa, Artificial Sequence
  Synthetic Light chain, clone:  E11
QSVLTQSPGTLSLSPGERATLSCRTSQILHSQYLAWYQQKRGQAPRLLIFRASTRATGIPERFSGSGSGRDFVLTISRLEPEDSAVYYCQQYETSWTFGQGTKVTVL

SEQ ID NO: 385 - protein, 107 aa, Artificial Sequence
  Synthetic Light chain, clone:  F12
QSVLTQDPVVSVALGQTVRITCQGDTLRTCYASWYQQRPRQAPILVIYGENNRPSGIPARFSGSSSGSTASLTITGAQAEDEGDYYCHCRDGLNHLVFGGGTKVTVL

SEQ ID NO: 386 - protein, 110 aa, Artificial Sequence
  Synthetic Light chain, clone:  C8
QSVLTQPPSVSAAPGQKVTISCSGSTSNIGKNFVSWYQHLPGTAPKLLIYDNYQRFSGIPDRFSGFKSGTSATLSITGLQTADEADYYCGTWDSSLSVVIFGGGTKLTVL

SEQ ID NO: 387 - protein, 107 aa, Artificial Sequence
  Synthetic Light chain, clone:  A8
QAGLTQSPDFQSVTPKERVTITCRASRYIGSNLHWYQQKPDQPPKLLIKLASQSFSGVPPRFSGGGSGTDFTLTINGLEAEDAATYYCHQTGSFPYTFGQGTKLTVL

SEQ ID NO: 388 - protein, 110 aa, Artificial Sequence
  Synthetic Light chain, clone:  B8
QAVLTQEPSLTVSPGGTVTLTCGSSTGAVTSGHSPFWFQQRPGQAPRTLIYDTSNKQSWTPARFSGSLLGGKAALTLSGAQPEDEAEYYCLLSYSGPRVVFGGGTKVTVL

SEQ ID NO: 389 - protein, 113 aa, Artificial Sequence
  Synthetic Light chain, clone:  F7
  misc_feature (27)..(27): Xaa can be any naturally occurring amino acid
QAVVTQSPDSLAVSLGERATISCKSSXSLLYRSNNKNYLAWYQQKPGQPPRLLISWASTRESGVPDRFSGSGSGTDFTLTVSRLRAEDAAVYYCQQSYRTPFSFGPGTKVTVL

SEQ ID NO: 390 - protein, 106 aa, Artificial Sequence
  Synthetic Light chain, clone:  B7
SYVLTQPLSVSVALGQTARISCGGANIANKNVHWYQLQPGQAPVLVIYRDSNRPSGIPERFSGSNSGNTATLTITRAQARDEADYYCQVWDSSSVIIGGGTKVTVL

SEQ ID NO: 391 - protein, 108 aa, Artificial Sequence
  Synthetic Light chain, clone:  G9
SYVLTQDPAVSVALGQTVRITCQGDSLRTYYASWYRQKPGQAPVLVFYGKDNRPSGIPDRFSGSSSGNTASLTITGAQAEDEADYYCKSRDSSAMRWVFGGGTKLTVL

SEQ ID NO: 392 - protein, 108 aa, Artificial Sequence
  Synthetic Light chain, clone:  A9
NFMLTQEPSLTVSPGGTVTLTCGSSTGAVTSGHYPYWFQQKPGQVPRTFIYDTHNRHSWTPVRFSGSLFGGKAALTLSGAQPEDEAEYYCLLYFNPTRVFGGGTKLTV

SEQ ID NO: 393 - protein, 110 aa, Artificial Sequence
  Synthetic Light chain, clone:  A11
NFMLTQPPSASASLGASVTLTCTLSSGYSNYKVDWYQQRPGKGPRFVMRVGTGGIVGSKGDGIPDRFSVLGSGLNRYLTIKNIQEEDESDYHCGADHGRVFGGGTKLTVL

SEQ ID NO: 394 - protein, 105 aa, Artificial Sequence
  Synthetic Light chain, clone:  E12
QPVLTQPPSVSVAPGKTARITCGGNNIGSKSVHWYHLRPGQAPVLVIYFDSDRPSGIPERFSGSNSGNTATLTISRVEAGDEADYYCQVWHSGVIFGGGTKLTVL

SEQ ID NO: 395 - protein, 106 aa, Artificial Sequence
  Synthetic Light chain, clone:  H7
QPVLTQSLDFQSVTPKEKVTITCRASQNIGNSLHWYQQKPNQSPKVLIKYASQSFSGVPSRFSGSGFGTDFTLTINSLEPEDAATYYCHQSRSSHTFGQGTKLTVL

SEQ ID NO: 396 - protein, 113 aa, Artificial Sequence
  Synthetic Light chain, clone:  A10
EIVLTQSPGNLSLSPGERATLSCTRCTGNIASHFVQWYQQRPGSSPTTVIFGNNQRPSGVSDRFSGSIDSSSNSASLTISRLKTEDEADYYCQSFDVYSHEVVFGGGTKLTVL

SEQ ID NO: 397 - protein, 113 aa, Artificial Sequence
  Synthetic Light chain, clone:  C11
QTVVTQTPVSLSVTPGQPASISCKSSQSLLNSDDGKTYLYWYLQRPGQPPHLLIYEVSKRFSGVPDRFSGSGSGTDFTLRISRVEAEDVGVFYCMQSTHFPFTFGPGTKVTVL

SEQ ID NO: 398 - protein, 107 aa, Artificial Sequence
  Synthetic Light chain, clone:  D10
NIQMTQSPVSLSASLGDTVSITCQASHDISNYLNWYQQKPGKAPKLLIYDASHLEAGVPSRFRGSGSGTDFTLTINRLEPEDFAVYYCQQYDSPPWTFGQGTKLTVL

SEQ ID NO: 399 - protein, 108 aa, Artificial Sequence
  Synthetic Light chain, clone:  D12
DVVLTQSPGTMSLSPGERATLSCRASQSVSRTYLAWHQQKPGQAPRLLIYGASSRAAGIPDRFSGSGSGTDFTLSISRLEPEDFAVYYCQQHDTSQWTFGQGTKLTVL

SEQ ID NO: 400 - protein, 112 aa, Artificial Sequence
  Synthetic Light chain, clone:  C7
DIVMTQTPLSLSVTPGQPASISCKSSQSLLHSDGKTHLFWYLQRPGQSPQLLIYEVSGRFSGVSERFSGSGSGTDFTLKISRVEAEDVGVYYCMQGLHIPHTFGQGTKVEIK

SEQ ID NO: 401 - protein, 111 aa, Artificial Sequence
  Synthetic Light chain, clone:  D7
DIVMTQSPLSLPVTLGQPASISCRSSHSLVHSDGNIYLNWYHQRPGQSPRRLIYSVSKRDSGVPDRFSGSGSRTDFTLKISRVEAEDVGVYFCMQSTHQWTFGQGTKVEIK

SEQ ID NO: 402 - protein, 107 aa, Artificial Sequence
  Synthetic Light chain, clone:  C9
  misc_feature (75)..(75): Xaa can be any naturally occurring amino acid
VIWMTQSPSTVSASVGDRVTITCRASQSISSWLAWYQQKPGKAPNLLIYEASRLESGIPSRFSGSGSGTEFTLTXSSLQPDDFATYYCQQYDSYSRTFGQGTKVAIK

SEQ ID NO: 403 - protein, 106 aa, Artificial Sequence
  Synthetic Light chain, clone:  C12
DVVMTQSPSSLSASVGDRVTITCRTSQGIRNYLSWYQQKPAKAPKLLIHGASGLQSGVPSRFSGSGSGTNFTLTISSLQPEDFATYYCQQSFSMRTFGQGTKVEIK

SEQ ID NO: 404 - protein, 114 aa, Artificial Sequence
  Synthetic Light chain, clone:  D8
EIVMTQSPGTLTLSPGEGATLSCRASQSVTSNYLAWYQQRPGASSLQSGQAPRLLIYDASNRATGIPDRFSGSGFGTDFTLTISRLEPEDFAVYYCQQYVNSRTFGQGTKVEIK

SEQ ID NO: 405 - protein, 106 aa, Artificial Sequence
  Synthetic Light chain, clone:  D9
EIVMTQSPVTLSVSPGERATLSCRASQSVSSKLAWYQQKPGQAPRLLIYGASTRATGIPARFSGSGSGTEFTLTISSLQSEDFAIYYCQQYNDFFTFGPGTKVDIK

SEQ ID NO: 406 - protein, 111 aa, Artificial Sequence
  Synthetic Light chain, clone:  G7
EIVLTQTPLSSPVTLGQPASISCRSSESPVHSDGNIYLSWLHQRPGQPPRLLLYKISNRMSGVPDRFSGSGAGTDFTLKISRVEAEDVGVYYCMQATQFPSFGQGTKLEIK

SEQ ID NO: 407 - protein, 108 aa, Artificial Sequence
  Synthetic Light chain, clone:  G11
EIVLTQSPGTLSLSPGEGATLSCRASQSVSSRNLAWYQQKPGQAPRLLIYGGSIRASGTSTRFSGSGSGTDFTLTINRLEPEDFAVYYCQQYGDSVFTFGPGTKVDIK

SEQ ID NO: 408 - protein, 107 aa, Artificial Sequence
  Synthetic Light chain, clone:  F9
NIQMTQSPSSLSASVGDRVNITCRASDNIGNYLNWYQHKPGKAPTVLIYAASTLHYGVPSRFSGRGSGTDFTVTISSLQPEDSATYYCQQSYSTPRTFGQGTRVELK

SEQ ID NO: 409 - protein, 108 aa, Artificial Sequence
  Synthetic Light chain, clone:  E9
AIQMTQSPSSLSASVGDRVTITCRASESISNYLNWYQQKPGKAPKLLLSAASRLQSGVPSRFSGSGSGTDFTLTITSLQPEDLATYYCQESYSTLLYTFGQGTKLEIK

SEQ ID NO: 410 - protein, 108 aa, Artificial Sequence
  Synthetic Light chain, clone:  B1
SYELTQPPSVSVAPGKTASITCGGNNIGYDSVHWYQQKPGQAPVLVVFDDSDRPSGIPERFSGSNSGNTATLTISRVEAGDEADYYCQVWESGSEHYVFGTGTQLTVL

SEQ ID NO: 411 - protein, 108 aa, Artificial Sequence
  Synthetic Light chain, clone:  E6
LPVLTQPPSVSVAPGQTARISCGGNNIGATTVHWYQHRPGQAPVSVIFYDNDRPSGIPERFSGSNSGNTATLTISRVEAGDEADYYCQVWESTSDHPTFGGGTQLTVL

SEQ ID NO: 412 - protein, 108 aa, Artificial Sequence
  Synthetic Light chain, clone:  F3
QSVLTQPPSVSVAPGKTARITCGGNNIGSKSVHWYQQKPGQAPVLVIYYDSDRPSGIPERFSGSNSGNTATLTISRVEAGDEADYYCQVWDSSSDHWVFGGGTKLTVL

SEQ ID NO: 413 - protein, 109 aa, Artificial Sequence
  Synthetic Light chain, clone:  H4
SYELTQSPSVSVPPGQTARITCGGNNIVSKGVHWYQQRPGQAPVLVVYDDSDRPSGIPERFAGFNSGNTATLTISRVEAGDEADYYCQVWDSSSGHRGVFGGGTKVTVL

SEQ ID NO: 414 - protein, 108 aa, Artificial Sequence
  Synthetic Light chain, clone:  H5
SYELTQPPSVSMAPGKTARITCGGNNLGSKIVHWYQQKPGQAPVVVIYSDRDRPSGVPERFSGSNSGNSATLTISGVEAGDEADYYCQVWDSATDHVVFGGGTKLTVL

SEQ ID NO: 415 - protein, 108 aa, Artificial Sequence
  Synthetic Light chain, clone:  B5
SYELTQPPSVSVAPGQTATITCAGNNIGGKSVQWYQQKPGQAPVVVVYDDYGRPSGIPERVSGSNSGNTATLTLTRVEAGDEADYYCQVWDSDRHHVVFGGGTKLTVL

SEQ ID NO: 416 - protein, 108 aa, Artificial Sequence
  Synthetic Light chain, clone:  G6
  misc_feature (75)..(75): Xaa can be any naturally occurring amino acid
  misc_feature (78)..(78): Xaa can be any naturally occurring amino acid
  misc_feature (104)..(104): Xaa can be any naturally occurring amino acid
QLVLTQPPSVSVSPGQTASITCSGDNLGHTNACWYQQNPGQSPVLVIYQDTKRPSGIPERFSGSNSGNPATLTIXRVXAGDEANYYCQVWDINDDYAVFGTGTXLTVL

SEQ ID NO: 417 - protein, 104 aa, Artificial Sequence
  Synthetic Light chain, clone:  C1
QSVLTQSPGTLSLSPGERATLSCTASQSVSSTYLTWYQQKPGQAPRLLIYGASSRATGIPDRFSGSGSGTDFTLTISRLEPEDFAVYYCQQYVSSPPMYTFGQL

SEQ ID NO: 418 - protein, 107 aa, Artificial Sequence
  Synthetic Light chain, clone:  F1
  misc_feature (38)..(38): Xaa can be any naturally occurring amino acid
  misc_feature (45)..(45): Xaa can be any naturally occurring amino acid
  misc_feature (61)..(61): Xaa can be any naturally occurring amino acid
  misc_feature (65)..(65): Xaa can be any naturally occurring amino acid
  misc_feature (82)..(82): Xaa can be any naturally occurring amino acid
DIQMTQSPSTLSASVGDRVTISCRASQNIDYDLAWYQXKPGKAPXLLIYGASNLEGGVPSXFSGXGSGTEFTLTISSLQPDXSATYYCQQYVTYPLTFGQGTRLEIK

SEQ ID NO: 419 - protein, 111 aa, Artificial Sequence
  Synthetic Light chain, clone:  A3
AIQMTQSPSSLSASVGDRVTMTCQASQVIDKYVNWYRQRPGKAPELLIYGASTLESGVPSRFSGSGSGTQFTFSITSVQPEDFATYICQQYDSVPLTFGPGTILDVKRTVA

SEQ ID NO: 420 - protein, 110 aa, Artificial Sequence
  Synthetic Light chain, clone:  B4
DIQLTQSPSSLSASIGDRVTITCQASQDIFHYLNWFQQKPGKAPKLLIYEASNLETGVPSRFSGSGSVTDFTFTISSLQPEDIATYYCQQYEDLPSFGGGTKVDIKRTVA

SEQ ID NO: 421 - protein, 108 aa, Artificial Sequence
  Synthetic Light chain, clone:  B6
EIVLTQSPGTLSLSPGERATLSCRASQSFGSNYLAWYQHKPGQAPRLLIFAASNRATGIPDRFTGSASGTDFTLTINRVEPEDLAVYYCQQYGSFPYSFGQGTKLEIK

SEQ ID NO: 422 - protein, 111 aa, Artificial Sequence
  Synthetic Light chain, clone:  F2
NIQMTQSPSSLSASVGDRVTITCQASQFIHIYLNWYQQKLGKAPKLLIYGASNLERGVPSRFSGRGSETDFTFTIDSLQPEDIATYFCQQYQNPPFTFGGGTKVEINGTVA

SEQ ID NO: 423 - protein, 111 aa, Artificial Sequence
  Synthetic Light chain, clone:  D3
AIRMTQSPSSLSASIGDRISVTCRASQDVGIYVAWFQQKPGKPPRSLIYAASYLQTAVPPKFRGSGSGTDFTLTISDLQPDDFATYYCQQYKTFPHTFGQGTKLDFKRTVA

SEQ ID NO: 424 - protein, 107 aa, Artificial Sequence
  Synthetic Light chain, clone:  G2
VIWMTQSPSTLSASVGDRVTITCRASQDINTWLAWYQQKPGKAPKLLMFKVSTLESGDFSRFSGSGSGTEFTLTVSSLQPDDSAIYYCQQYHSYPYTFGQGTRLEIK

SEQ ID NO: 425 - protein, 107 aa, Artificial Sequence
  Synthetic Light chain, clone:  A4
DVVMTQSPSSLSASVGDRVTITCQASQDISNWLNWYQQKPGKAPKLLIYEASNLETGVPSRFSGSGSGTDFTFTISSLQPEDIATYYCQQYNNVLRTFGQGTKVEIK

SEQ ID NO: 426 - protein, 106 aa, Artificial Sequence
  Synthetic Light chain, clone:  G4
  misc_feature (6)..(6): Xaa can be any naturally occurring amino acid
  misc_feature (79)..(79): Xaa can be any naturally occurring amino acid
EIVMTXSPATLSVSPGERVTLSCRVSQNVFSDLAWYQRKTGQSPRLLIHGASTRATGIPTRFSGSGSGTEFTLTISSLXSDDFAVYYCQQYNKWPTFGQGTKVEIK

SEQ ID NO: 427 - protein, 112 aa, Artificial Sequence
  Synthetic Light chain, clone:  D5
AIQLTQSPSSLSASVGDRVNITCRASDNIGNYLNWYQHKPGKAPTVLIYAASTLHYGVPSRFSGRGSGTDFTVTISSLRSDDFAVYYCQQYYNWPPWTFGQGTTVDIKRTVA

SEQ ID NO: 428 - protein, 106 aa, Artificial Sequence
  Synthetic Light chain, clone:  A1
EIVLTQSPATLSLSPGERATLSCRASQSVSSFLAWYQQKPGQAPRLLIFEASTRATGISARFSGSGSGTDFTLTISTLEPEDFAVYYCQQRSNGVTFGQGTRLEIK

SEQ ID NO: 429 - protein, 111 aa, Artificial Sequence
  Synthetic Light chain, clone:  H2
DIQMTQSPSTLSASVGDTVTITCRATESISIWLAWYQQEPGKAPNLLVSQASSLKTGVPSRFSASGSGTEFTLTISSLHPDDFATYVCQHYHTYPFTFGPGTKVDMKRTVA

SEQ ID NO: 430 - protein, 116 aa, Artificial Sequence
  Synthetic Light chain, clone:  E2
  misc_feature (11)..(11): Xaa can be any naturally occurring amino acid
EIVLTQSPDSXAVSLGERATINCKSSQSVLYSSNNKNYLAWYQQKPGQPPRLLIYWASTRESGVPDRFSGSGSGTDFTLTISRLQAEDVAVYYCQQYYLTPTFTVTFGQGTKLEIK

SEQ ID NO: 431 - protein, 111 aa, Artificial Sequence
  Synthetic Light chain, clone:  F4
DIQLTQSPSSVSASVGDRVTITCRASQDISSWLAWYQQKPGKAPKFLIYRATNLQSGVPSRFSGSGSGTDFTLTISSLQPGDFATYYCQQTNTFPLTFGGGTKVEVKRTVA

SEQ ID NO: 432 - protein, 113 aa, Artificial Sequence
  Synthetic Light chain, clone:  C5
DIVMTQSPDSLAVSLGERATINCKSSQSVLYSSNNRNYLAWYQKKPGQPPKLLFYWASTRESGVSDRFSGSGSGTDFTLTISSLQAEDVAVYYCQQYHTTPYTFGQGTKLEIK

SEQ ID NO: 433 - protein, 111 aa, Artificial Sequence
  Synthetic Light chain, clone:  E5
VIWMTQSPSSLSASVGDRVSITCRASQTFTSHLNWYQQKPGQPPKLLIFAASNLQSGVPSRFSGSGSGTDFTLTINGLQATDFATYYCQQSFSSPWTFGQGTTVDVKGTVA

SEQ ID NO: 434 - protein, 111 aa, Artificial Sequence
  Synthetic Light chain, clone:  F6
DIQMTQSPSSLSASVGDRVTITCRASQSVNVYLNWYQQKPGKAPKLLIYSASTLQSGVPSRFTGSGSRTDFTLTINGLQPEDFATYYCQQSFTTLVTFGPGTRVDVTRTVA

SEQ ID NO: 435 - protein, 111 aa, Artificial Sequence
  Synthetic Light chain, clone:  G5
DIQMTQSPSSLSASVGDRVTITCRASQDISSSLAWYQQKPGKAPKPLIYDASTLQTGVPSRFSGRASGTDFTLTIDSLQPEDFATYCCQQFNSYPLSFGGGTKVELKRTVA

SEQ ID NO: 436 - protein, 116 aa, Artificial Sequence
  Synthetic Light chain, clone:  A5
SYELTQPPSASASLGASVTLTCTVSSGYRSYEVDWFQQRPGKGPRFVMRVGTGGIVGSRGDGIPDRFSVWGSGLNRYLTIEDIQEEDESDYYCGADHGSGSNLVYVFGTGTKVTVL

SEQ ID NO: 437 - protein, 116 aa, Artificial Sequence
  Synthetic Light chain, clone:  D6
QLVLTQPPSASASLGASVTLTCTLSSDYSSYNVDWYQQRPGMGPRFLMRVGTGGIVGSRGDGIPDRFSVKGSGLNRYLTIKNIQEEDESDYYCGADHGSGSDFVYVFGIGTKLTVL

SEQ ID NO: 438 - protein, 110 aa, Artificial Sequence
  Synthetic Light chain, clone:  E4
QSVLTQPPSASGTPGQRVTISCSGSSTNIGSNAVNWYQQLPRTAPKLLIYTNNQRPSGVPDRFSGSKSGTSASLAISGLQSEDEANYYCAAWDDSLNGPVFGGGTQLTVL

SEQ ID NO: 439 - protein, 110 aa, Artificial Sequence
  Synthetic Light chain, clone:  F5
QSVLTQPPSASGTPGQTVIISCSGGGSNIGSNFGYWYQQFPGTAPKLLIYTTDRRPSGVPDRFSGSKSGTTASLAISGLRSEDEADYYCAAWDDRLSGPVFGGGTQLTVL

SEQ ID NO: 440 - protein, 112 aa, Artificial Sequence
  Synthetic Light chain, clone:  G1
QTVVTQPPSVSGTPGQRVTISCSGSSSNIGSNSVDWYQQFPGSAPKLLIYTTNQRPSGVPDRFSGSKSGTSASLAISGLRSEDEADYYCATWDDDLSNPKWVFGGGTKLTVL

SEQ ID NO: 441 - protein, 112 aa, Artificial Sequence
  Synthetic Light chain, clone:  E3
DIVMTQSPLSLPVTPGEPASISCRSSQSLLHSNGYNFLDWYLQKPGQSPQLLIYLGSNRASGVPDRFSGSGSGTDFTLKISRVEAEDVGIYYCMQALQTSWTFGQGTKLEIK

SEQ ID NO: 442 - protein, 114 aa, Artificial Sequence
  Synthetic Light chain, clone:  A2
DICRIRPLIRLTIGTITIYNYNGCCDDTVSTLPARHPWTAGLHLQSPRRLMYQVSTRDSGVPDRFSGSGSGTDFTLRISRVEAEDVGVYYCMQGTHWPYTFGQGTKLEIRRTVA

SEQ ID NO: 443 - protein, 112 aa, Artificial Sequence
  Synthetic Light chain, clone:  D1
DIVMTQTPLSLSVTPGQPAAISCKSSQSLVHRDGKTYLYWYLQKPGHSPQLLVYEASSRFSGVPDRISGSASGTQFTLNISRVEAEDVGLYYCMQSRNLPKTFGQGTKVEIK

SEQ ID NO: 444 - protein, 108 aa, Artificial Sequence
  Synthetic Light chain, clone:  C4
SYELTQPTSLSASPGASASLTCTLSSGFNVVSYNIYWYQQKPGSPPQYLLRYRSDSDRHQGSGVPSRFSGSKDASANAGILVISALQSDDEADYYCMVWYSAWVFGGG

SEQ ID NO: 445 - protein, 107 aa, Artificial Sequence
  Synthetic Light chain, clone:  E1
SYELTQPLSVSVALGQTATITCAGNNIGTYYVHWYQQRPGQAPVLVMYRDTNRPSGISDRFSGSNSGDTATLTICGVQVGDEADYYCHVLDSSTIVIFGGGTQLTVL

SEQ ID NO: 446 - protein, 108 aa, Artificial Sequence
  Synthetic Light chain, clone:  A6
QSVLTQSPATLSVSPGERASLSCRASQSVSSNLAWYQQKPGQAPRLLIYGASTRATGIPARFSGSGSGTEFTLTISSLQSEDFAVYYCHQYNNWPLYTFGQGTKLTVL

SEQ ID NO: 447 - protein, 108 aa, Artificial Sequence
  Synthetic Light chain, clone:  H1
QSVLTQDPAVPVALGQTVRITCQGDSLRTYYASWYQQKPGQAPLLVIYGKNTRPSGIPVRFSGSSSGNTASLTITGAQAEDEADYYCNSRDSSGYLLLFGTGTKLTVL

SEQ ID NO: 448 - protein, 109 aa, Artificial Sequence
  Synthetic Light chain, clone:  B2
QAVLTQEPSLTVSPGGTVTLTCGSSTGAVTSGHYPYWFQQKPGQAPRTLIYDASNKHSWTPARFSGSLLGGKAALTLSGAQPEDEAEYYCLLSYSGAGVFGTGTKVTVL

SEQ ID NO: 449 - protein, 111 aa, Artificial Sequence
  Synthetic Light chain, clone:  C2
DIQMTQSPSSLSASVGDRVAIACRPSQDIGTDLGWYQQKPGKAPKLLIFDSSTLQSGVPSRFSGSLSGTDFILTITNLQPEDFATYYCLQDYSFPYTFGQGTKLQIKRTVA

SEQ ID NO: 450 - protein, 106 aa, Artificial Sequence
  Synthetic Light chain, clone:  G3
SYVLTQPPSVSVSPGQTASITCSGDELKYKYTCWYHQKPGQSPVLLIYQDTKRPSGIPERFSGSRSENTATLTISGTQAMDEADYYCQAWDSSHAVFGRGTQLTVL

SEQ ID NO: 451 - protein, 107 aa, Artificial Sequence
  Synthetic Light chain, clone:  H3
HSYVLTQPPSVSVFPGQTARITCSGSTFPKLYSFWYQQKTGQAPLLVIYKDTERPSGIPERFSGSTSGTTVTLIISGVQPEDDADYYCQSEDSRGPVFGGGTKVTVL

SEQ ID NO: 452 - protein, 112 aa, Artificial Sequence
  Synthetic Light chain, clone:  D4
GVVMTQTPLSSLVTLGQPASISCRSSESVVHDDGNTYLSWLQQRPGQPPRLLIYKISNRFSGVPDRFSGSGAGTDFTLKISRVEPEDVGVYYCVQATHFPVTFGGGTRVEIK

SEQ ID NO: 453 - protein, 111 aa, Artificial Sequence
  Synthetic Light chain, clone:  C6
QSALTQPASVSASPGQSVTISCTGTSDDVGRYDYVSWYQQHPGGAPKLILYDVNRRPSGVSDRFSGSKSANKASLTISGLQADDEGDYYCCSYTTGSTLYLFGTGTQLTVL

SEQ ID NO: 454 - DNA, 18 bp, Artificial Sequence
  Synthetic Oligonucleotide:  FR3 Reverse
cgcacagtaatacacggc

SEQ ID NO: 455 - DNA, 46 bp, Artificial Sequence
  Synthetic Oligonucleotide:  VH1a
caattactatttacaattacaatgcaggtkcagctggtgcagtctg

SEQ ID NO: 456 - DNA, 46 bp, Artificial Sequence
  Synthetic Oligonucleotide:  VH1b
caattactatttacaattacaatgcaggtccagcttgtgcagtctg

SEQ ID NO: 457 - DNA, 46 bp, Artificial Sequence
  Synthetic Oligonucleotide:  VH1c
caattactatttacaattacaatgsaggtccagctggtacagtctg

SEQ ID NO: 458 - DNA, 46 bp, Artificial Sequence
  Synthetic Oligonucleotide:  VH1d
caattactatttacaattacaatgcaratgcagctggtgcagtctg

SEQ ID NO: 459 - DNA, 46 bp, Artificial Sequence
  Synthetic Oligonucleotide:  VH2
caattactatttacaattacaatgcagrtcaccttgaaggagtctg

SEQ ID NO: 460 - DNA, 46 bp, Artificial Sequence
  Synthetic Oligonucleotide:  VH3a
caattactatttacaattacaatggargtgcagctggtggagtctg

SEQ ID NO: 461 - DNA, 46 bp, Artificial Sequence
  Synthetic Oligonucleotide:  VH3b
caattactatttacaattacaatgcaggtgcagctggtggagtctg

SEQ ID NO: 462 - DNA, 46 bp, Artificial Sequence
  Synthetic Oligonucleotide:  VH3c
caattactatttacaattacaatggaggtgcagctgttggagtctg

SEQ ID NO: 463 - DNA, 42 bp, Artificial Sequence
  Synthetic Oligonucleotide:  VH4a
caattactatttacaattacaatgcagstgcagctgcaggag

SEQ ID NO: 464 - DNA, 45 bp, Artificial Sequence
  Synthetic Oligonucleotide:  VH4b
caattactatttacaattacaatgcaggtgcagctacagcagtgg

SEQ ID NO: 465 - DNA, 46 bp, Artificial Sequence
  Synthetic Oligonucleotide:  VH5
caattactatttacaattacaatggargtgcagctggtgcagtctg

SEQ ID NO: 466 - DNA, 46 bp, Artificial Sequence
  Synthetic Oligonucleotide:  VH6
caattactatttacaattacaatgcaggtacagctgcagcagtcag

SEQ ID NO: 467 - DNA, 46 bp, Artificial Sequence
  Synthetic Oligonucleotide:  VH7
caattactatttacaattacaatgcaggtgcagctggtgcaatctg

SEQ ID NO: 468 - DNA, 42 bp, Artificial Sequence
  Synthetic Oligonucleotide:  T7TMVUTR
taatacgactcactatagggacaattactatttacaattaca

SEQ ID NO: 469 - DNA, 75 bp, Artificial Sequence
  Synthetic Oligonucleotide:  XB1511 FR3CDR3FR4 Reverse
tgaggagacggtgaccagggttccctggccccagtagctcctgtcgcccccatgtktcgcacagtaatacacggc

SEQ ID NO: 470 - DNA, 39 bp, Artificial Sequence
  Synthetic Oligonucleotide:  FR4 Cu3 Reverse
ggagacgagggggaaaagggttgaggagacggtgaccag

SEQ ID NO: 471 - DNA, 87 bp, Artificial Sequence
  Synthetic Oligonucleotide:  Y109
ttttttttttttttttttttaaatagcggatgctaaggacgacttgtcgtcgtcgtccttgtagtcggagacgagggggaaaagggt

SEQ ID NO: 472 - DNA, 21 bp, Artificial Sequence
  Synthetic Oligonucleotide:  Ck1
caactgctcatcagatggcgg

SEQ ID NO: 473 - DNA, 21 bp, Artificial Sequence
  Synthetic Oligonucleotide:  Cl1
cagtgtggccttgttggcttg

SEQ ID NO: 474 - DNA, 21 bp, Artificial Sequence
  Synthetic Oligonucleotide:  Ck2
agatggtgcagccacagttcg

SEQ ID NO: 475 - DNA, 41 bp, Artificial Sequence
  Synthetic Oligonucleotide:  Jl1-3Ck2
agatggtgcagccacagttcgtagacggtsascttggtccc

SEQ ID NO: 476 - DNA, 41 bp, Artificial Sequence
  Synthetic Oligonucleotide:  Jl7Ck2
agatggtgcagccacagttcggagacggtcagctgggtgcc

SEQ ID NO: 477 - DNA, 42 bp, Artificial Sequence; identical to SEQ ID NO: 468
  Synthetic Oligonucleotide:  T7TMVUTR

SEQ ID NO: 478 - DNA, 42 bp, Artificial Sequence
  Synthetic Oligonucleotide:  UTRVk1a
caattactatttacaattacaatgracatccagatgacccag

SEQ ID NO: 479 - DNA, 42 bp, Artificial Sequence
  Synthetic Oligonucleotide:  UTRVk1b
caattactatttacaattacaatggmcatccagttgacccag

SEQ ID NO: 480 - DNA, 42 bp, Artificial Sequence
  Synthetic Oligonucleotide:  UTRVk1c
caattactatttacaattacaatggccatccrgatgacccag

SEQ ID NO: 481 - DNA, 42 bp, Artificial Sequence
  Synthetic Oligonucleotide:  UTRVk1d
caattactatttacaattacaatggtcatctggatgacccag

SEQ ID NO: 482 - DNA, 42 bp, Artificial Sequence
  Synthetic Oligonucleotide:  UTRVk2a
caattactatttacaattacaatggatattgtgatgacccag

SEQ ID NO: 483 - DNA, 42 bp, Artificial Sequence
  Synthetic Oligonucleotide:  UTRVk2b
caattactatttacaattacaatggatrttgtgatgactcag

SEQ ID NO: 484 - DNA, 42 bp, Artificial Sequence
  Synthetic Oligonucleotide:  UTRVk3a
caattactatttacaattacaatggaaattgtgttgacrcag

SEQ ID NO: 485 - DNA, 42 bp, Artificial Sequence
  Synthetic Oligonucleotide:  UTRVk3b
caattactatttacaattacaatggaaatagtgatgacgcag

SEQ ID NO: 486 - DNA, 42 bp, Artificial Sequence
  Synthetic Oligonucleotide:  UTRVk3c
caattactatttacaattacaatggaaattgtaatgacacag

SEQ ID NO: 487 - DNA, 42 bp, Artificial Sequence
  Synthetic Oligonucleotide:  UTRVk4a
caattactatttacaattacaatggacatcgtgatgacccag

SEQ ID NO: 488 - DNA, 42 bp, Artificial Sequence
  Synthetic Oligonucleotide:  UTRVk5a
caattactatttacaattacaatggaaacgacactcacgcag

SEQ ID NO: 489 - DNA, 42 bp, Artificial Sequence
  Synthetic Oligonucleotide:  UTRVk6a
caattactatttacaattacaatggaaattgtgctgactcag

SEQ ID NO: 490 - DNA, 42 bp, Artificial Sequence
  Synthetic Oligonucleotide:  UTRVk6b
caattactatttacaattacaatggatgttgtgatgacacag

SEQ ID NO: 491 - DNA, 42 bp, Artificial Sequence
  Synthetic Oligonucleotide:  UTRVL1a
caattactatttacaattacaatgcagtctgtgctgackcag

SEQ ID NO: 492 - DNA, 42 bp, Artificial Sequence
  Synthetic Oligonucleotide:  UTRVL1b
caattactatttacaattacaatgcagtctgtgytgacgcag

SEQ ID NO: 493 - DNA, 42 bp, Artificial Sequence
  Synthetic Oligonucleotide:  UTRVL2
caattactatttacaattacaatgcagtctgccctgactcag

SEQ ID NO: 494 - DNA, 42 bp, Artificial Sequence
  Synthetic Oligonucleotide:  UTRVL3a
caattactatttacaattacaatgtcctatgwgctgactcag

SEQ ID NO: 495 - DNA, 42 bp, Artificial Sequence
  Synthetic Oligonucleotide:  UTRVL3b
caattactatttacaattacaatgtcctatgagctgacacag

SEQ ID NO: 496 - DNA, 42 bp, Artificial Sequence
  Synthetic Oligonucleotide:  UTRVL3c
caattactatttacaattacaatgtcttctgagctgactcag

SEQ ID NO: 497 - DNA, 42 bp, Artificial Sequence
  Synthetic Oligonucleotide:  UTRVL3d
caattactatttacaattacaatgtcctatgagctgatgcag

SEQ ID NO: 498 - DNA, 42 bp, Artificial Sequence
  Synthetic Oligonucleotide:  UTRVL4
caattactatttacaattacaatgcagcytgtgctgactcaa

SEQ ID NO: 499 - DNA, 42 bp, Artificial Sequence
  Synthetic Oligonucleotide:  UTRVL5
caattactatttacaattacaatgcagsctgtgctgactcag

SEQ ID NO: 500 - DNA, 42 bp, Artificial Sequence
  Synthetic Oligonucleotide:  UTRVL6
caattactatttacaattacaatgaattttatgctgactcag

SEQ ID NO: 501 - DNA, 42 bp, Artificial Sequence
  Synthetic Oligonucleotide:  UTRVL7
caattactatttacaattacaatgcagrctgtggtgactcag

SEQ ID NO: 502 - DNA, 42 bp, Artificial Sequence
  Synthetic Oligonucleotide:  UTRVL8
caattactatttacaattacaatgcagactgtggtgacccag

SEQ ID NO: 503 - DNA, 42 bp, Artificial Sequence
  Synthetic Oligonucleotide:  UTRVL4/9
caattactatttacaattacaatgcwgcctgtgctgactcag

SEQ ID NO: 504 - DNA, 42 bp, Artificial Sequence
  Synthetic Oligonucleotide:  UTRVL10
caattactatttacaattacaatgcaggcagggctgactcag

SEQ ID NO: 505 - protein, 464 aa, Artificial Sequence
  Synthetic Antibody chain:  XB1511 IgG1
GWSLILLFLVAVATRVLSQVQLVQSGAEVKKPGSSVKVSCKASGGTFSSYAISWVRQAPGQGLEWMGGIIPIFGTANYAQKFQGRVTITADESTSTAYMELSSLRSEDTAVYYCAIHGGDRSYWGQGTLVTVSSASTKGPSVFPLAPSSKSTSGGTAALGCLVKDYFPEPVTVSWNSGALTSGVHTFPAVLQSSGLYSLSSVVTVPSSSLGTQTYICNVNHKPSNTKVDKKVEPKSCDKTHTCPPCPAPELLGGPSVFLFPPKPKDTLMISRTPEVTCVVVDVSHEDPEVKFNWYVDGVEVHNAKTKPREEQYNSTYRVVSVLTVLHQDWLNGKEYKCKVSNKALPAPIEKTISKAKGQPREPQVYTLPPSRDELTKNQVSLTCLVKGFYPSDIAVEWESNGQPENNYKTTPPVLDSDGSFFLYSKLTVDKSRWQQGNVFSCSVMHEALHNHYTQKSLSLSPGK

SEQ ID NO: 506 - protein, 262 aa, Artificial Sequence
  Synthetic Antibody chain:  D8 Ckappa
DFQVQIISFLLISASVIMSRGEIVMTQSPGTLTLSPGEGATLSCRASQSVTSNYLAWYQQRPGQAPRLLIYDASNRATGIPDRFSGSGFGTDFTLTISRLEPEDFAVYYCQQYVNSRTFGQGTKVEIKRTVAAPSVFIFPPSDEQLKSGTKVEIKRTVAAPSVFIFPPSDEQLKSGTASVVCLLNNFYPREAKVQWKVDNALQSGNSQESVTEQDSKDSTYSLSSTLTLSKADYEKHKVYACEVTHQGLSSPVTKSFNRGEC

SEQ ID NO: 507 - protein, 464 aa, Artificial Sequence
  Synthetic Antibody chain:  XB2202 IgG1
GWSLILLFLVAVATRVLSQVQLVQSGAEVKKPGSSVRVSCKASGGTFSRHAISWVRQAPGQGLEWIGGILPILKTPNYAQRFQGRVTINADESTSTVYMEMSSLRSEDTAVYYCATHGGDRSYWGQGTLVTVSSASTKGPSVFPLAPSSKSTSGGTAALGCLVKDYFPEPVTVSWNSGALTSGVHTFPAVLQSSGLYSLSSVVTVPSSSLGTQTYICNVNHKPSNTKVDKKVEPKSCDKTHTCPPCPAPELLGGPSVFLFPPKPKDTLMISRTPEVTCVVVDVSHEDPEVKFNWYVDGVEVHNAKTKPREEQYNSTYRVVSVLTVLHQDWLNGKEYKCKVSNKALPAPIEKTISKAKGQPREPQVYTLPPSRDELTKNQVSLTCLVKGFYPSDIAVEWESNGQPENNYKTTPPVLDSDGSFFLYSKLTVDKSRWQQGNVFSCSVMHEALHNHYTQKSLSLSPGK

SEQ ID NO: 508 - protein, 262 aa, Artificial Sequence
  Synthetic Antibody chain:  A4 Ckappa
DFQVQIISFLLISASVIMSRGDVVMTQSPSSLSASVGDRVTITCQASQDISNWLNWYQQKPGKAPKLLIYEASNLETGVPSRFSGSGSGTDFTFTISSLQPEDIATYYCQQYNNVLRTFGQGTKVEIKRTVAAPSVFIFPPSDEQLKSGTKVEIKRTVAAPSVFIFPPSDEQLKSGTASVVCLLNNFYPREAKVQWKVDNALQSGNSQESVTEQDSKDSTYSLSSTLTLSKADYEKHKVYACEVTHQGLSSPVTKSFNRGEC